European Patent Specification EP 3 189 069 B1, published October 23, 2024. Title: APOE MIMETIC PEPTIDES AND HIGHER POTENCY TO CLEAR PLASMA CHOLESTEROL. Applicant: LIPIMETIX DEVELOPMENT, LLC Anantharamaiah, G.M. Goldberg, Dennis. The sequence listing filed with the application follows.

SEQUENCE LISTING (661 sequences)

SEQ ID NO: 1 - protein, 28 aa, Artificial Sequence
  synthetic construct; ApoE mimetic
LRKLRKRLLRDWLKAFYDKVAEKLKEAF

SEQ ID NO: 2 - protein, 28 aa, Artificial Sequence
  synthetic construct; reverse analog of ApoE mimetic
RLLRKRLKRLDWLKAFYDKVAEKLKEAF

SEQ ID NO: 3 - protein, 28 aa, Artificial Sequence
  synthetic construct; reverse analog of ApoE mimetic
LRKLRKRLLRFAEKLKEAVKDYFAKLWD

SEQ ID NO: 4 - protein, 10 aa, Artificial Sequence
  synthetic construct; receptor binding domain of human Apo E
LRKLRKRLLR

SEQ ID NO: 5 - protein, 18 aa, Artificial Sequence
  synthetic construct; lipid-associating peptide
DWLKAFYDKVAEKLKEAF

SEQ ID NO: 6 - protein, 10 aa, Artificial Sequence
  synthetic construct; analog of receptor binding domain of human Apo E
LRRLRRRLLR

SEQ ID NO: 7 - protein, 10 aa, Artificial Sequence
  synthetic construct; Rat ApoE mimetic
LRKMRKRLMR

SEQ ID NO: 8 - protein, 10 aa, Artificial Sequence
  synthetic construct; Bovine Apo E mimetic
LRKLPKRLLR

SEQ ID NO: 9 - protein, 10 aa, Artificial Sequence
  synthetic construct; Pig ApoE mimetic
LRNVRKRLVR

SEQ ID NO: 10 - protein, 10 aa, Artificial Sequence
  synthetic construct; Dog ApoE mimetic
MRKLRKRVLR

SEQ ID NO: 11 - protein, 10 aa, Artificial Sequence
  synthetic construct; R modified ApoE mimetic
LRRLRRRLLR

SEQ ID NO: 12 - protein, 10 aa, Artificial Sequence
  synthetic construct; F modified ApoE mimetic
LRKLRKRFFR

SEQ ID NO: 13 - protein, 9 aa, Artificial Sequence
  synthetic construct; ApoB mimetic
RLTRKRGLK

SEQ ID NO: 14 - protein, 18 aa, Artificial Sequence
  synthetic construct; class A peptide
DWFKAFYDKVAEKLKEAF

SEQ ID NO: 15 - protein, 18 aa, Artificial Sequence
  synthetic construct; class A peptide
DWLKAFYDKVAEKFKEAF

SEQ ID NO: 16 - protein, 18 aa, Artificial Sequence
  synthetic construct; class A peptide
DWFKAFYDKVAEKFKEAF

SEQ ID NO: 17 - protein, 18 aa, Artificial Sequence
  synthetic construct; class A peptide
DWLKAFYDKVFEKFKEFF

SEQ ID NO: 18 - protein, 18 aa, Artificial Sequence
  synthetic construct; class A peptide
DWLKAFYDKFFEKFKEFF

SEQ ID NO: 19 - protein, 18 aa, Artificial Sequence
  synthetic construct; class A peptide
DWFKAFYDKFFEKFKEFF

SEQ ID NO: 20 - protein, 18 aa, Artificial Sequence
  synthetic construct; class A peptide
DWLKAFYDKVAEKLKEFF

SEQ ID NO: 21 - protein, 18 aa, Artificial Sequence
  synthetic construct; class A peptide
DWLKAFYDKVFEKLKEFF

SEQ ID NO: 22 - protein, 18 aa, Artificial Sequence
  synthetic construct; class A peptide
DWLKAFYDKVFEKFKEFF

SEQ ID NO: 23 - protein, 18 aa, Artificial Sequence
  synthetic construct; class A peptide
EWLKLFYEKVLEKFKEAF

SEQ ID NO: 24 - protein, 19 aa, Artificial Sequence
  synthetic construct; class A peptide
EWLKAFYIDKVAEKFKEAF

SEQ ID NO: 25 - protein, 19 aa, Artificial Sequence
  synthetic construct; class A peptide
EEWLKAFYDKVAEKLKEFF

SEQ ID NO: 26 - protein, 18 aa, Artificial Sequence
  synthetic construct; class A peptide
EWLKAFYDKVFEKFKEAF

SEQ ID NO: 27 - protein, 18 aa, Artificial Sequence
  synthetic construct; class A peptide
EWLKAFYDKVFEKLKEFF

SEQ ID NO: 28 - protein, 18 aa, Artificial Sequence
  synthetic construct; class A peptide
EWLKAFYDKVAEKFKEFF

SEQ ID NO: 29 - protein, 18 aa, Artificial Sequence
  synthetic construct; class A peptide
EWLKAFYDKVFEKFKEFF

SEQ ID NO: 30 - protein, 14 aa, Artificial Sequence
  synthetic construct; class A peptide
AFYDKVAEKLKEAF

SEQ ID NO: 31 - protein, 14 aa, Artificial Sequence
  synthetic construct; class A peptide
AFYDKVAEKFKEAF

SEQ ID NO: 32 - protein, 14 aa, Artificial Sequence
  synthetic construct; class A peptide
AFYDKVAEKFKEAF

SEQ ID NO: 33 - protein, 14 aa, Artificial Sequence
  synthetic construct; class A peptide
AFYDKFFEKFKEFF

SEQ ID NO: 34 - protein, 14 aa, Artificial Sequence
  synthetic construct; class A peptide
AFYDKFFEKFKEFF

SEQ ID NO: 35 - protein, 14 aa, Artificial Sequence
  synthetic construct; class A peptide
AFYDKVAEKFKEAF

SEQ ID NO: 36 - protein, 14 aa, Artificial Sequence
  synthetic construct; class A peptide
AFYDKVAEKLKEFF

SEQ ID NO: 37 - protein, 14 aa, Artificial Sequence
  synthetic construct; class A peptide
AFYDKVFEKFKEAF

SEQ ID NO: 38 - protein, 14 aa, Artificial Sequence
  synthetic construct; class A peptide
AFYDKVFEKLKEFF

SEQ ID NO: 39 - protein, 14 aa, Artificial Sequence
  synthetic construct; class A peptide
AFYDKVAEKFKEFF

SEQ ID NO: 40 - protein, 14 aa, Artificial Sequence
  synthetic construct; class A peptide
KAFYDKVFEKFKEF

SEQ ID NO: 41 - protein, 14 aa, Artificial Sequence
  synthetic construct; class A peptide
LFYEKVLEKFKEAF

SEQ ID NO: 42 - protein, 14 aa, Artificial Sequence
  synthetic construct; class A peptide
AFYDKVAEKFKEAF

SEQ ID NO: 43 - protein, 14 aa, Artificial Sequence
  synthetic construct; class A peptide
AFYDKVAEKLKEFF

SEQ ID NO: 44 - protein, 14 aa, Artificial Sequence
  synthetic construct; class A peptide
AFYDKVFEKFKEAF

SEQ ID NO: 45 - protein, 14 aa, Artificial Sequence
  synthetic construct; class A peptide
AFYDKVFEKLKEFF

SEQ ID NO: 46 - protein, 14 aa, Artificial Sequence
  synthetic construct; class A peptide
AFYDKVAEKFKEFF

SEQ ID NO: 47 - protein, 14 aa, Artificial Sequence
  synthetic construct; class A peptide
AFYDKVFEKFKEFF

SEQ ID NO: 48 - protein, 18 aa, Artificial Sequence
  synthetic construct; class A peptide
DWLKALYDKVAEKLKEAL

SEQ ID NO: 49 - protein, 18 aa, Artificial Sequence
  synthetic construct; class A peptide
DWFKAFYEKVAEKLKEFF

SEQ ID NO: 50 - protein, 18 aa, Artificial Sequence
  synthetic construct; class A peptide
DWFKAFYEKFFEKFKEFF

SEQ ID NO: 51 - protein, 18 aa, Artificial Sequence
  synthetic construct; class A peptide
EWLKALYEKVAEKLKEAL

SEQ ID NO: 52 - protein, 18 aa, Artificial Sequence
  synthetic construct; class A peptide
EWLKAFYEKVAEKLKEAF

SEQ ID NO: 53 - protein, 18 aa, Artificial Sequence
  synthetic construct; class A peptide
EWFKAFYEKVAEKLKEFF

SEQ ID NO: 54 - protein, 18 aa, Artificial Sequence
  synthetic construct; class A peptide
EWLKAFYEKVFEKFKEFF

SEQ ID NO: 55 - protein, 18 aa, Artificial Sequence
  synthetic construct; class A peptide
EWLKAFYEKFFEKFKEFF

SEQ ID NO: 56 - protein, 18 aa, Artificial Sequence
  synthetic construct; class A peptide
EWFKAFYEKFFEKFKEFF

SEQ ID NO: 57 - protein, 18 aa, Artificial Sequence
  synthetic construct; class A peptide
DFLKAWYDKVAEKLKEAW

SEQ ID NO: 58 - protein, 18 aa, Artificial Sequence
  synthetic construct; class A peptide
EFLKAWYEKVAEKLKEAW

SEQ ID NO: 59 - protein, 18 aa, Artificial Sequence
  synthetic construct; class A peptide
DFWKAWYDKVAEKLKEWW

SEQ ID NO: 60 - protein, 18 aa, Artificial Sequence
  synthetic construct; class A peptide
EFWKAWYEKVAEKLKEWW

SEQ ID NO: 61 - protein, 18 aa, Artificial Sequence
  synthetic construct; class A peptide
DKLKAFYDKVFEWAKEAF

SEQ ID NO: 62 - protein, 18 aa, Artificial Sequence
  synthetic construct; class A peptide
DKWKAVYDKFAEAFKEFL

SEQ ID NO: 63 - protein, 18 aa, Artificial Sequence
  synthetic construct; class A peptide
EKLKAFYEKVFEWAKEAF

SEQ ID NO: 64 - protein, 18 aa, Artificial Sequence
  synthetic construct; class A peptide
EKWKAVYEKFAEAFKEFL

SEQ ID NO: 65 - protein, 18 aa, Artificial Sequence
  synthetic construct; class A peptide
DWLKAFVDKFAEKFKEAY

SEQ ID NO: 66 - protein, 18 aa, Artificial Sequence
  synthetic construct; class A peptide
EKWKAVYEKFAEAFKEFL

SEQ ID NO: 67 - protein, 18 aa, Artificial Sequence
  synthetic construct; class A peptide
DWLKAFVYDKVFKLKEFF

SEQ ID NO: 68 - protein, 18 aa, Artificial Sequence
  synthetic construct; class A peptide
EWLKAFVYEKVFKLKEFF

SEQ ID NO: 69 - protein, 18 aa, Artificial Sequence
  synthetic construct; class A peptide
DWLRAFYDKVAEKLKEAF

SEQ ID NO: 70 - protein, 18 aa, Artificial Sequence
  synthetic construct; class A peptide
EWLRAFYEKVAEKLKEAF

SEQ ID NO: 71 - protein, 18 aa, Artificial Sequence
  synthetic construct; class A peptide
DWLKAFYDRVAEKLKEAF

SEQ ID NO: 72 - protein, 18 aa, Artificial Sequence
  synthetic construct; class A peptide
EWLKAFYERVAEKLKEAF

SEQ ID NO: 73 - protein, 18 aa, Artificial Sequence
  synthetic construct; class A peptide
DWLKAFYDKVAERLKEAF

SEQ ID NO: 74 - protein, 18 aa, Artificial Sequence
  synthetic construct; class A peptide
EWLKAFYEKVAERLKEAF

SEQ ID NO: 75 - protein, 18 aa, Artificial Sequence
  synthetic construct; class A peptide
DWLKAFYDKVAEKLREAF

SEQ ID NO: 76 - protein, 18 aa, Artificial Sequence
  synthetic construct; class A peptide
EWLKAFYEKVAEKLREAF

SEQ ID NO: 77 - protein, 18 aa, Artificial Sequence
  synthetic construct; class A peptide
DWLKAFYDRVAERLKEAF

SEQ ID NO: 78 - protein, 18 aa, Artificial Sequence
  synthetic construct; class A peptide
EWLKAFYERVAERLKEAF

SEQ ID NO: 79 - protein, 18 aa, Artificial Sequence
  synthetic construct; class A peptide
DWLRAFYDKVAEKLREAF

SEQ ID NO: 80 - protein, 18 aa, Artificial Sequence
  synthetic construct; class A peptide
EWLRAFYEKVAEKLREAF

SEQ ID NO: 81 - protein, 18 aa, Artificial Sequence
  synthetic construct; class A peptide
DWLRAFYDRVAEKLKEAF

SEQ ID NO: 82 - protein, 18 aa, Artificial Sequence
  synthetic construct; class A peptide
EWLRAFYERVAEKLKEAF

SEQ ID NO: 83 - protein, 18 aa, Artificial Sequence
  synthetic construct; class A peptide
DWLKAFYDKVAERLREAF

SEQ ID NO: 84 - protein, 18 aa, Artificial Sequence
  synthetic construct; class A peptide
EWLKAFYEKVAERLREAF

SEQ ID NO: 85 - protein, 18 aa, Artificial Sequence
  synthetic construct; class A peptide
DWLRAFYDKVAERLKEAF

SEQ ID NO: 86 - protein, 18 aa, Artificial Sequence
  synthetic construct; class A peptide
EWLRAFYEKVAERLKEAF

SEQ ID NO: 87 - protein, 37 aa, Artificial Sequence
  synthetic construct; class A peptide
DWLKAFYDKVAEKLKEAFPDWLKAFYDKVAEKLKEAF

SEQ ID NO: 88 - protein, 37 aa, Artificial Sequence
  synthetic construct; class A peptide
DWLKAFYDKVAEKLKEFFPDWLKAFYDKVAEKLKEFF

SEQ ID NO: 89 - protein, 37 aa, Artificial Sequence
  synthetic construct; class A peptide
DWFKAFYDKVAEKLKEAFPDWFKAFYDKVAEKLKEAF

SEQ ID NO: 90 - protein, 37 aa, Artificial Sequence
  synthetic construct; class A peptide
DKLKAFYDKVFEWAKEAFPDKLKAFYDKVFEWLKEAF

SEQ ID NO: 91 - protein, 37 aa, Artificial Sequence
  synthetic construct; class A peptide
DKWKAVYDKFAEAFKEFLPDKWKAVYDKFAEAFKEFL

SEQ ID NO: 92 - protein, 37 aa, Artificial Sequence
  synthetic construct; class A peptide
DWFKAFYDKVAEKFKEAFPDWFKAFYDKVAEKFKEAF

SEQ ID NO: 93 - protein, 37 aa, Artificial Sequence
  synthetic construct; class A peptide
DWLKAFVYDKVFKLKEFFPDWLKAFVYDKVFKLKEFF

SEQ ID NO: 94 - protein, 37 aa, Artificial Sequence
  synthetic construct; class A peptide
DWLKAFYDKFAEKFKEFFPDWLKAFYDKFAEKFKEFF

SEQ ID NO: 95 - protein, 18 aa, Artificial Sequence
  synthetic construct; class A peptide
EWFKAFYEKVAEKFKEAF

SEQ ID NO: 96 - protein, 14 aa, Artificial Sequence
  synthetic construct; class A peptide
DWFKAFYDKVAEKF

SEQ ID NO: 97 - protein, 14 aa, Artificial Sequence
  synthetic construct; class A peptide
FKAFYDKVAEKFKE

SEQ ID NO: 98 - protein, 14 aa, Artificial Sequence
  synthetic construct; class A peptide
FKAFYEKVAEKFKE

SEQ ID NO: 99 - protein, 14 aa, Artificial Sequence
  synthetic construct; class A peptide
FKAFYDKVAEKFKE

SEQ ID NO: 100 - protein, 14 aa, Artificial Sequence
  synthetic construct; class A peptide
FKAFYEKVAEKFKE

SEQ ID NO: 101 - protein, 18 aa, Artificial Sequence
  synthetic construct; class A peptide
DWFKAFYDKVAEKFKEAF

SEQ ID NO: 102 - protein, 18 aa, Artificial Sequence
  synthetic construct; class A peptide
EWFKAFYEKVAEKFKEAF

SEQ ID NO: 103 - protein, 14 aa, Artificial Sequence
  synthetic construct; class A peptide
AFYDKVAEKFKEAF

SEQ ID NO: 104 - protein, 14 aa, Artificial Sequence
  synthetic construct; class A peptide
DWFKAFYDKVAEKF

SEQ ID NO: 105 - protein, 18 aa, Artificial Sequence
  synthetic construct; class A peptide
DWLKAFYDKVFEKFKEFF

SEQ ID NO: 106 - protein, 18 aa, Artificial Sequence
  synthetic construct; class A peptide
DWLKAFYDKVFEKFKEFF

SEQ ID NO: 107 - protein, 18 aa, Artificial Sequence
  synthetic construct; class A peptide
EWLKAFYEKVFEKFKEFF

SEQ ID NO: 108 - protein, 18 aa, Artificial Sequence
  synthetic construct; class A peptide
EWLKAFYEKVFEKFKEFF

SEQ ID NO: 109 - protein, 14 aa, Artificial Sequence
  synthetic construct; class A peptide
AFYDKVFEKFKEFF

SEQ ID NO: 110 - protein, 14 aa, Artificial Sequence
  synthetic construct; class A peptide
AFYDKVFEKFKEFF

SEQ ID NO: 111 - protein, 14 aa, Artificial Sequence
  synthetic construct; class A peptide
AFYEKVFEKFKEFF

SEQ ID NO: 112 - protein, 14 aa, Artificial Sequence
  synthetic construct; class A peptide
AFYEKVFEKFKEFF

SEQ ID NO: 113 - protein, 14 aa, Artificial Sequence
  synthetic construct; class A peptide
DWLKAFYDKVFEKF

SEQ ID NO: 114 - protein, 14 aa, Artificial Sequence
  synthetic construct; class A peptide
DWLKAFYDKVFEKF

SEQ ID NO: 115 - protein, 14 aa, Artificial Sequence
  synthetic construct; class A peptide
EWLKAFYEKVFEKF

SEQ ID NO: 116 - protein, 14 aa, Artificial Sequence
  synthetic construct; class A peptide
EWLKAFYEKVFEKF

SEQ ID NO: 117 - protein, 14 aa, Artificial Sequence
  synthetic construct; class A peptide
LKAFYDKVFEKFKE

SEQ ID NO: 118 - protein, 14 aa, Artificial Sequence
  synthetic construct; class A peptide
LKAFYDKVFEKFKE

SEQ ID NO: 119 - protein, 14 aa, Artificial Sequence
  synthetic construct; class A peptide
LKAFYEKVFEKFKE

SEQ ID NO: 120 - protein, 14 aa, Artificial Sequence
  synthetic construct; class A peptide
LKAFYEKVFEKFKE

SEQ ID NO: 121 - protein, 18 aa, Artificial Sequence
  synthetic construct; modified class A peptide
DKWKAVYDKFAEAFKEFL

SEQ ID NO: 122 - protein, 18 aa, Artificial Sequence
  synthetic construct; modified class A peptide
DKLKAFYDKVFEWAKEAF

SEQ ID NO: 123 - protein, 18 aa, Artificial Sequence
  synthetic construct; Class A amphipathic helical peptides
EWFKAFYEKVADKFKDAF

SEQ ID NO: 124 - protein, 18 aa, Artificial Sequence
  synthetic construct; Class A amphipathic helical peptides
EWFKAFYDKVADKFKEAF

SEQ ID NO: 125 - protein, 18 aa, Artificial Sequence
  synthetic construct; Class A amphipathic helical peptides
DWFKAFYEKVADKFKEAF

SEQ ID NO: 126 - protein, 18 aa, Artificial Sequence
  synthetic construct; Class A amphipathic helical peptides
DWFKAFYEKVAEKFKDAF

SEQ ID NO: 127 - protein, 18 aa, Artificial Sequence
  synthetic construct; Class A amphipathic helical peptides
DFWKAFYDKVAEKFKEAF

SEQ ID NO: 128 - protein, 18 aa, Artificial Sequence
  synthetic construct; Class A amphipathic helical peptides
EFWKAFYEKVADKFKDAF

SEQ ID NO: 129 - protein, 18 aa, Artificial Sequence
  synthetic construct; Class A amphipathic helical peptides
EFWKAFYDKVADKFKEAF

SEQ ID NO: 130 - protein, 18 aa, Artificial Sequence
  synthetic construct; Class A amphipathic helical peptides
DFWKAFYEKVADKFKEAF

SEQ ID NO: 131 - protein, 18 aa, Artificial Sequence
  synthetic construct; Class A amphipathic helical peptides
DFWKAFYEKVAEKFKDAF

SEQ ID NO: 132 - protein, 18 aa, Artificial Sequence
  synthetic construct; Class A amphipathic helical peptides
DWFKAYFDKVAEKFKEAF

SEQ ID NO: 133 - protein, 18 aa, Artificial Sequence
  synthetic construct; Class A amphipathic helical peptides
EWFKAYFEKVADKFKDAF

SEQ ID NO: 134 - protein, 18 aa, Artificial Sequence
  synthetic construct; Class A amphipathic helical peptides
EWFKAYFDKVADKFKEAF

SEQ ID NO: 135 - protein, 18 aa, Artificial Sequence
  synthetic construct; Class A amphipathic helical peptides
DWFKAYFEKVADKFKEAF

SEQ ID NO: 136 - protein, 18 aa, Artificial Sequence
  synthetic construct; Class A amphipathic helical peptides
DWFKAYFEKVAEKFKDAF

SEQ ID NO: 137 - protein, 18 aa, Artificial Sequence
  synthetic construct; Class A amphipathic helical peptides
DWFKAFVDKYAEKFKEAF

SEQ ID NO: 138 - protein, 18 aa, Artificial Sequence
  synthetic construct; Class A amphipathic helical peptides
EWFKAFVEKYADKFKDAF

SEQ ID NO: 139 - protein, 18 aa, Artificial Sequence
  synthetic construct; Class A amphipathic helical peptides
EWFKAFVDKYADKFKEAF

SEQ ID NO: 140 - protein, 18 aa, Artificial Sequence
  synthetic construct; Class A amphipathic helical peptides
DWFKAFVEKYADKFKEAF

SEQ ID NO: 141 - protein, 18 aa, Artificial Sequence
  synthetic construct; Class A amphipathic helical peptides
DWFKAFVEKYAEKFKDAF

SEQ ID NO: 142 - protein, 18 aa, Artificial Sequence
  synthetic construct; Class A amphipathic helical peptides
DWFKAFYDKAVEKFKEAF

SEQ ID NO: 143 - protein, 18 aa, Artificial Sequence
  synthetic construct; Class A amphipathic helical peptides
EWFKAFYEKAVDKFKDAF

SEQ ID NO: 144 - protein, 18 aa, Artificial Sequence
  synthetic construct; Class A amphipathic helical peptides
EWFKAFYDKAVDKFKEAF

SEQ ID NO: 145 - protein, 18 aa, Artificial Sequence
  synthetic construct; Class A amphipathic helical peptides
DWFKAFYEKAVDKFKEAF

SEQ ID NO: 146 - protein, 18 aa, Artificial Sequence
  synthetic construct; Class A amphipathic helical peptides
DWFKAFYEKAVEKFKDAF

SEQ ID NO: 147 - protein, 18 aa, Artificial Sequence
  synthetic construct; Class A amphipathic helical peptides
DWFKAFYDKVFEKAKEAF

SEQ ID NO: 148 - protein, 18 aa, Artificial Sequence
  synthetic construct; Class A amphipathic helical peptides
EWFKAFYEKVFDKAKDAF

SEQ ID NO: 149 - protein, 18 aa, Artificial Sequence
  synthetic construct; Class A amphipathic helical peptides
EWFKAFYDKVFDKAKEAF

SEQ ID NO: 150 - protein, 18 aa, Artificial Sequence
  synthetic construct; Class A amphipathic helical peptides
DWFKAFYEKVFDKAKEAF

SEQ ID NO: 151 - protein, 18 aa, Artificial Sequence
  synthetic construct; Class A amphipathic helical peptides
DWFKAFYEKVFEKAKDAF

SEQ ID NO: 152 - protein, 18 aa, Artificial Sequence
  synthetic construct; Class A amphipathic helical peptides
DWFKAFYDKVAEKAKEFF

SEQ ID NO: 153 - protein, 18 aa, Artificial Sequence
  synthetic construct; Class A amphipathic helical peptides
EWFKAFYEKVADKAKDFF

SEQ ID NO: 154 - protein, 18 aa, Artificial Sequence
  synthetic construct; Class A amphipathic helical peptides
EWFKAFYDKVADKAKEFF

SEQ ID NO: 155 - protein, 18 aa, Artificial Sequence
  synthetic construct; Class A amphipathic helical peptides
DWFKAFYEKVADKAKEFF

SEQ ID NO: 156 - protein, 18 aa, Artificial Sequence
  synthetic construct; Class A amphipathic helical peptides
DWFKAFYEKVAEKAKDFF

SEQ ID NO: 157 - protein, 18 aa, Artificial Sequence
  synthetic construct; Class A amphipathic helical peptides
DWFKAFYDKVAEKFKEFA

SEQ ID NO: 158 - protein, 18 aa, Artificial Sequence
  synthetic construct; Class A amphipathic helical peptides
EWFKAFYEKVADKFKDFA

SEQ ID NO: 159 - protein, 18 aa, Artificial Sequence
  synthetic construct; Class A amphipathic helical peptides
EWFKAFYDKVADKFKEFA

SEQ ID NO: 160 - protein, 18 aa, Artificial Sequence
  synthetic construct; Class A amphipathic helical peptides
DWFKAFYEKVADKFKEFA

SEQ ID NO: 161 - protein, 18 aa, Artificial Sequence
  synthetic construct; Class A amphipathic helical peptides
DWFKAFYEKVAEKFKDFA

SEQ ID NO: 162 - protein, 18 aa, Artificial Sequence
  synthetic construct; Class A amphipathic helical peptides
DAFKAFYDKVAEKFKEWF

SEQ ID NO: 163 - protein, 18 aa, Artificial Sequence
  synthetic construct; Class A amphipathic helical peptides
EAFKAFYEKVADKFKDWF

SEQ ID NO: 164 - protein, 18 aa, Artificial Sequence
  synthetic construct; Class A amphipathic helical peptides
EAFKAFYDKVADKFKEWF

SEQ ID NO: 165 - protein, 18 aa, Artificial Sequence
  synthetic construct; Class A amphipathic helical peptides
DAFKAFYEKVADKFKEWF

SEQ ID NO: 166 - protein, 18 aa, Artificial Sequence
  synthetic construct; Class A amphipathic helical peptides
DAFKAFYEKVAEKFKDWF

SEQ ID NO: 167 - protein, 18 aa, Artificial Sequence
  synthetic construct; Class A amphipathic helical peptides
DAFKAFYDKVWEKFKEAF

SEQ ID NO: 168 - protein, 18 aa, Artificial Sequence
  synthetic construct; Class A amphipathic helical peptides
EAFKAFYEKVWDKFKDAF

SEQ ID NO: 169 - protein, 18 aa, Artificial Sequence
  synthetic construct; Class A amphipathic helical peptides
EAFKAFYDKVWDKFKEAF

SEQ ID NO: 170 - protein, 18 aa, Artificial Sequence
  synthetic construct; Class A amphipathic helical peptides
DAFKAFYEKVWDKFKEAF

SEQ ID NO: 171 - protein, 18 aa, Artificial Sequence
  synthetic construct; Class A amphipathic helical peptides
DAFKAFYEKVWEKFKDAF

SEQ ID NO: 172 - protein, 18 aa, Artificial Sequence
  synthetic construct; Class A amphipathic helical peptides
DYFKAFWDKVAEKFKEAF

SEQ ID NO: 173 - protein, 18 aa, Artificial Sequence
  synthetic construct; Class A amphipathic helical peptides
EYFKAFWEKVADKFKDAF

SEQ ID NO: 174 - protein, 18 aa, Artificial Sequence
  synthetic construct; Class A amphipathic helical peptides
EYFKAFWDKVADKFKEAF

SEQ ID NO: 175 - protein, 18 aa, Artificial Sequence
  synthetic construct; Class A amphipathic helical peptides
DYFKAFWEKVADKFKEAF

SEQ ID NO: 176 - protein, 18 aa, Artificial Sequence
  synthetic construct; Class A amphipathic helical peptides
DYFKAFWEKVAEKFKDAF

SEQ ID NO: 177 - protein, 18 aa, Artificial Sequence
  synthetic construct; Class A amphipathic helical peptides
DWAKAFYDKVAEKFKEFF

SEQ ID NO: 178 - protein, 18 aa, Artificial Sequence
  synthetic construct; Class A amphipathic helical peptides
EWAKAFYEKVADKFKDFF

SEQ ID NO: 179 - protein, 18 aa, Artificial Sequence
  synthetic construct; Class A amphipathic helical peptides
EWAKAFYDKVADKFKEFF

SEQ ID NO: 180 - protein, 18 aa, Artificial Sequence
  synthetic construct; Class A amphipathic helical peptides
DWAKAFYEKVADKFKEFF

SEQ ID NO: 181 - protein, 18 aa, Artificial Sequence
  synthetic construct; Class A amphipathic helical peptides
DWAKAFYEKVAEKFKDFF

SEQ ID NO: 182 - protein, 18 aa, Artificial Sequence
  synthetic construct; Class A amphipathic helical peptides
DWFKAAYDKVAEKFKEFF

SEQ ID NO: 183 - protein, 18 aa, Artificial Sequence
  synthetic construct; Class A amphipathic helical peptides
EWFKAAYEKVADKFKDFF

SEQ ID NO: 184 - protein, 18 aa, Artificial Sequence
  synthetic construct; Class A amphipathic helical peptides
EWFKAAYDKVADKFKEFF

SEQ ID NO: 185 - protein, 18 aa, Artificial Sequence
  synthetic construct; Class A amphipathic helical peptides
DWFKAAYEKVADKFKEFF

SEQ ID NO: 186 - protein, 18 aa, Artificial Sequence
  synthetic construct; Class A amphipathic helical peptides
DWFKAAYEKVAEKFKDFF

SEQ ID NO: 187 - protein, 18 aa, Artificial Sequence
  synthetic construct; Class A amphipathic helical peptides
DWFKAFADKVAEKFKEYF

SEQ ID NO: 188 - protein, 18 aa, Artificial Sequence
  synthetic construct; Class A amphipathic helical peptides
EWFKAFAEKVADKFKDYF

SEQ ID NO: 189 - protein, 18 aa, Artificial Sequence
  synthetic construct; Class A amphipathic helical peptides
EWFKAFADKVADKFKEYF

SEQ ID NO: 190 - protein, 18 aa, Artificial Sequence
  synthetic construct; Class A amphipathic helical peptides
DWFKAFAEKVADKFKEYF

SEQ ID NO: 191 - protein, 18 aa, Artificial Sequence
  synthetic construct; Class A amphipathic helical peptides
DWFKAFAEKVAEKFKDYF

SEQ ID NO: 192 - protein, 18 aa, Artificial Sequence
  synthetic construct; Class A amphipathic helical peptides
DWFKAFYDKAAEKFKEVF

SEQ ID NO: 193 - protein, 18 aa, Artificial Sequence
  synthetic construct; Class A amphipathic helical peptides
EWFKAFYEKAADKFKDVF

SEQ ID NO: 194 - protein, 18 aa, Artificial Sequence
  synthetic construct; Class A amphipathic helical peptides
EWFKAFYDKAADKFKEVF

SEQ ID NO: 195 - protein, 18 aa, Artificial Sequence
  synthetic construct; Class A amphipathic helical peptides
DWFKAFYEKAADKFKEVF

SEQ ID NO: 196 - protein, 18 aa, Artificial Sequence
  synthetic construct; Class A amphipathic helical peptides
DWFKAFYEKAAEKFKDVF

SEQ ID NO: 197 - protein, 18 aa, Artificial Sequence
  synthetic construct; Class A amphipathic helical peptides
DWYKAFFDKVAEKFKEAF

SEQ ID NO: 198 - protein, 18 aa, Artificial Sequence
  synthetic construct; Class A amphipathic helical peptides
EWYKAFFEKVADKFKDAF

SEQ ID NO: 199 - protein, 18 aa, Artificial Sequence
  synthetic construct; Class A amphipathic helical peptides
EWYKAFFDKVADKFKEAF

SEQ ID NO: 200 - protein, 18 aa, Artificial Sequence
  synthetic construct; Class A amphipathic helical peptides
DWYKAFFEKVADKFKEAF

SEQ ID NO: 201 - protein, 18 aa, Artificial Sequence
  synthetic construct; Class A amphipathic helical peptides
DWYKAFFEKVAEKFKDAF

SEQ ID NO: 202 - protein, 18 aa, Artificial Sequence
  synthetic construct; Class A amphipathic helical peptides
DWVKAFYDKFAEKFKEAF

SEQ ID NO: 203 - protein, 18 aa, Artificial Sequence
  synthetic construct; Class A amphipathic helical peptides
EWVKAFYEKFADKFKDAF

SEQ ID NO: 204 - protein, 18 aa, Artificial Sequence
  synthetic construct; Class A amphipathic helical peptides
EWVKAFYDKFADKFKEAF

SEQ ID NO: 205 - protein, 18 aa, Artificial Sequence
  synthetic construct; Class A amphipathic helical peptides
DWVKAFYEKFADKFKEAF

SEQ ID NO: 206 - protein, 18 aa, Artificial Sequence
  synthetic construct; Class A amphipathic helical peptides
DWVKAFYEKFAEKFKDAF

SEQ ID NO: 207 - protein, 18 aa, Artificial Sequence
  synthetic construct; Class A amphipathic helical peptides
DWFKAFFDKVAEKYKEAF

SEQ ID NO: 208 - protein, 18 aa, Artificial Sequence
  synthetic construct; Class A amphipathic helical peptides
EWFKAFFEKVADKYKDAF

SEQ ID NO: 209 - protein, 18 aa, Artificial Sequence
  synthetic construct; Class A amphipathic helical peptides
EWFKAFFDKVADKYKEAF

SEQ ID NO: 210 - protein, 18 aa, Artificial Sequence
  synthetic construct; Class A amphipathic helical peptides
DWFKAFFEKVADKYKEAF

SEQ ID NO: 211 - protein, 18 aa, Artificial Sequence
  synthetic construct; Class A amphipathic helical peptides
DWFKAFFEKVADKYKEAF

SEQ ID NO: 212 - protein, 18 aa, Artificial Sequence
  synthetic construct; Class A amphipathic helical peptides
DWFKAFFDKVAEKFKEAY

SEQ ID NO: 213 - protein, 18 aa, Artificial Sequence
  synthetic construct; Class A amphipathic helical peptides
EWFKAFFEKVADKFKDAY

SEQ ID NO: 214 - protein, 18 aa, Artificial Sequence
  synthetic construct; Class A amphipathic helical peptides
EWFKAFFDKVADKFKEAY

SEQ ID NO: 215 - protein, 18 aa, Artificial Sequence
  synthetic construct; Class A amphipathic helical peptides
DWFKAFFEKVADKFKEAY

SEQ ID NO: 216 - protein, 18 aa, Artificial Sequence
  synthetic construct; Class A amphipathic helical peptides
DWFKAFFEKVAEKFKDAY

SEQ ID NO: 217 - protein, 18 aa, Artificial Sequence
  synthetic construct; Class A amphipathic helical peptides
DWFKAFYDKFAEKFKEAV

SEQ ID NO: 218 - protein, 18 aa, Artificial Sequence
  synthetic construct; Class A amphipathic helical peptides
EWFKAFYEKFADKFKDAV

SEQ ID NO: 219 - protein, 18 aa, Artificial Sequence
  synthetic construct; Class A amphipathic helical peptides
EWFKAFYDKFADKFKEAV

SEQ ID NO: 220 - protein, 18 aa, Artificial Sequence
  synthetic construct; Class A amphipathic helical peptides
DWFKAFYEKFADKFKEAV

SEQ ID NO: 221 - protein, 18 aa, Artificial Sequence
  synthetic construct; Class A amphipathic helical peptides
DWFKAFYEKFAEKFKDAV

SEQ ID NO: 222 - protein, 18 aa, Artificial Sequence
  synthetic construct; Class A amphipathic helical peptides
DKFKAFYDKVAEKFWEAF

SEQ ID NO: 223 - protein, 18 aa, Artificial Sequence
  synthetic construct; Class A amphipathic helical peptides
EKFKAFYEKVADKFWDAF

SEQ ID NO: 224 - protein, 18 aa, Artificial Sequence
  synthetic construct; Class A amphipathic helical peptides
EKFKAFYDKVADKFWEAF

SEQ ID NO: 225 - protein, 18 aa, Artificial Sequence
  synthetic construct; Class A amphipathic helical peptides
DKFKAFYEKVADKFWEAF

SEQ ID NO: 226 - protein, 18 aa, Artificial Sequence
  synthetic construct; Class A amphipathic helical peptides
DKFKAFYEKVAEKFWDAF

SEQ ID NO: 227 - protein, 18 aa, Artificial Sequence
  synthetic construct; Class A amphipathic helical peptides
DKWKAFYDKVAEKFFEAF

SEQ ID NO: 228 - protein, 18 aa, Artificial Sequence
  synthetic construct; Class A amphipathic helical peptides
EKWKAFYEKVADKFFDAF

SEQ ID NO: 229 - protein, 18 aa, Artificial Sequence
  synthetic construct; Class A amphipathic helical peptides
EKWKAFYDKVADKFFEAF

SEQ ID NO: 230 - protein, 18 aa, Artificial Sequence
  synthetic construct; Class A amphipathic helical peptides
DKWKAFYEKVADKFFEAF

SEQ ID NO: 231 - protein, 18 aa, Artificial Sequence
  synthetic construct; Class A amphipathic helical peptides
DKWKAFYEKVAEKFFDAF

SEQ ID NO: 232 - protein, 18 aa, Artificial Sequence
  synthetic construct; Class A amphipathic helical peptides
DKFKAFYDKWAEVFKEAF

SEQ ID NO: 233 - protein, 18 aa, Artificial Sequence
  synthetic construct; Class A amphipathic helical peptides
EKFKAFYEKWADVFKDAF

SEQ ID NO: 234 - protein, 18 aa, Artificial Sequence
  synthetic construct; Class A amphipathic helical peptides
EKFKAFYDKWADVFKEAF

SEQ ID NO: 235 - protein, 18 aa, Artificial Sequence
  synthetic construct; Class A amphipathic helical peptides
DKFKAFYEKWADVFKEAF

SEQ ID NO: 236 - protein, 18 aa, Artificial Sequence
  synthetic construct; Class A amphipathic helical peptides
DKFKAFYEKWAEVFKDAF

SEQ ID NO: 237 - protein, 18 aa, Artificial Sequence
  synthetic construct; Class A amphipathic helical peptides
DKFKAFYDKVAEFWKEAF

SEQ ID NO: 238 - protein, 18 aa, Artificial Sequence
  synthetic construct; Class A amphipathic helical peptides
EKFKAFYEKVADFWKDAF

SEQ ID NO: 239 - protein, 18 aa, Artificial Sequence
  synthetic construct; Class A amphipathic helical peptides
EKFCAFYDKVADFWKEAF

SEQ ID NO: 240 - protein, 18 aa, Artificial Sequence
  synthetic construct; Class A amphipathic helical peptides
DKFKAFYEKVADFWKEAF

SEQ ID NO: 241 - protein, 18 aa, Artificial Sequence
  synthetic construct; Class A amphipathic helical peptides
DKFKAFYEKVAEFWKDAF

SEQ ID NO: 242 - protein, 18 aa, Artificial Sequence
  synthetic construct; Class A amphipathic helical peptides
FAEKFKEAVKDYFAKFWD

SEQ ID NO: 243 - protein, 18 aa, Artificial Sequence
  synthetic construct; Class A amphipathic helical peptides
FADKFKDAVKEYFAKFWE

SEQ ID NO: 244 - protein, 18 aa, Artificial Sequence
  synthetic construct; Class A amphipathic helical peptides
FADKFKEAVKDYFAKFWE

SEQ ID NO: 245 - protein, 18 aa, Artificial Sequence
  synthetic construct; Class A amphipathic helical peptides
FAEKFKDAVKEYFAKFWD

SEQ ID NO: 246 - protein, 18 aa, Artificial Sequence
  synthetic construct; Class A amphipathic helical peptides
FAEKFKDAVKDYFAKFWE

SEQ ID NO: 247 - protein, 18 aa, Artificial Sequence
  synthetic construct; Class A amphipathic helical peptides
FWEKFKEAVKDYFAKFAD

SEQ ID NO: 248 - protein, 18 aa, Artificial Sequence
  synthetic construct; Class A amphipathic helical peptides
FWDKFKDAVKEYFAKFAE

SEQ ID NO: 249 - protein, 18 aa, Artificial Sequence
  synthetic construct; Class A amphipathic helical peptides
FADKFKEAVKDYFAKFWE

SEQ ID NO: 250 - protein, 18 aa, Artificial Sequence
  synthetic construct; Class A amphipathic helical peptides
FAEKFKDAVKEYFAKFWD

SEQ ID NO: 251 - protein, 18 aa, Artificial Sequence
  synthetic construct; Class A amphipathic helical peptides
FAEKFKDAVKDYFAKFWE

SEQ ID NO: 252 - protein, 18 aa, Artificial Sequence
  synthetic construct; Class A amphipathic helical peptides
FFEKFKEAVKDYFAKAWD

SEQ ID NO: 253 - protein, 18 aa, Artificial Sequence
  synthetic construct; Class A amphipathic helical peptides
FFDKFKDAVKEYFAKAWE

SEQ ID NO: 254 - protein, 18 aa, Artificial Sequence
  synthetic construct; Class A amphipathic helical peptides
FFDKFKEAVKDYFAKAWE

SEQ ID NO: 255 - protein, 18 aa, Artificial Sequence
  synthetic construct; Class A amphipathic helical peptides
FFEKFKDAVKEYFAKAWD

SEQ ID NO: 256 - protein, 18 aa, Artificial Sequence
  synthetic construct; Class A amphipathic helical peptides
FFEKFKDAVKDYFAKAWE

SEQ ID NO: 257 - protein, 18 aa, Artificial Sequence
  synthetic construct; Class A amphipathic helical peptides
FAEKAKEFVKDYFAKFWD

SEQ ID NO: 258 - protein, 18 aa, Artificial Sequence
  synthetic construct; Class A amphipathic helical peptides
FADKAKDFVKEYFAKFWE

SEQ ID NO: 259 - protein, 18 aa, Artificial Sequence
  synthetic construct; Class A amphipathic helical peptides
FADKAKEFVKDYFAKFWE

SEQ ID NO: 260 - protein, 18 aa, Artificial Sequence
  synthetic construct; Class A amphipathic helical peptides
FAEKAKDFVKEYFAKFWD

SEQ ID NO: 261 - protein, 18 aa, Artificial Sequence
  synthetic construct; Class A amphipathic helical peptides
FAEKAKDFVKDYFAKFWE

SEQ ID NO: 262 - protein, 18 aa, Artificial Sequence
  synthetic construct; Class A amphipathic helical peptides
FAEKFKEVAKDYFAKFWD

SEQ ID NO: 263 - protein, 18 aa, Artificial Sequence
  synthetic construct; Class A amphipathic helical peptides
FADKFKDVAKEYFAKFWE

SEQ ID NO: 264 - protein, 18 aa, Artificial Sequence
  synthetic construct; Class A amphipathic helical peptides
FADKFKEVAKDYFAKFWE

SEQ ID NO: 265 - protein, 18 aa, Artificial Sequence
  synthetic construct; Class A amphipathic helical peptides
FAEKFKDVAKEYFAKFWD

SEQ ID NO: 266 - protein, 18 aa, Artificial Sequence
  synthetic construct; Class A amphipathic helical peptides
FAEKFKDVAKDYFAKFWE

SEQ ID NO: 267 - protein, 18 aa, Artificial Sequence
  synthetic construct; Class A amphipathic helical peptides
FADKFKEAYKDVFAKFWE

SEQ ID NO: 268 - protein, 18 aa, Artificial Sequence
  synthetic construct; Class A amphipathic helical peptides
FAEKFKDAYKEVFAKFWD

SEQ ID NO: 269 - protein, 18 aa, Artificial Sequence
  synthetic construct; Class A amphipathic helical peptides
FAEKFKDAYKDVFAKFWE

SEQ ID NO: 270 - protein, 18 aa, Artificial Sequence
  synthetic construct; Class A amphipathic helical peptides
FAEKFKEAVKDFYAKFWD

SEQ ID NO: 271 - protein, 18 aa, Artificial Sequence
  synthetic construct; Class A amphipathic helical peptides
FADKFKDAVKEFYAKFWE

SEQ ID NO: 272 - protein, 18 aa, Artificial Sequence
  synthetic construct; Class A amphipathic helical peptides
FADKFKEAVKDFYAKFWE

SEQ ID NO: 273 - protein, 18 aa, Artificial Sequence
  synthetic construct; Class A amphipathic helical peptides
FAEKFKDAVKEFYAKFWD

SEQ ID NO: 274 - protein, 18 aa, Artificial Sequence
  synthetic construct; Class A amphipathic helical peptides
FAEKFKDAVKDFYAKFWE

SEQ ID NO: 275 - protein, 18 aa, Artificial Sequence
  synthetic construct; Class A amphipathic helical peptides
FAEKFWEAVKDYFAKFKD

SEQ ID NO: 276 - protein, 18 aa, Artificial Sequence
  synthetic construct; Class A amphipathic helical peptides
FADKFWDAVKEYFAKFKE

SEQ ID NO: 277 - protein, 18 aa, Artificial Sequence
  synthetic construct; Class A amphipathic helical peptides
FADKFWEAVKDYFAKFKE

SEQ ID NO: 278 - protein, 18 aa, Artificial Sequence
  synthetic construct; Class A amphipathic helical peptides
FAEKFWDAVKEYFAKFKD

SEQ ID NO: 279 - protein, 18 aa, Artificial Sequence
  synthetic construct; Class A amphipathic helical peptides
FAEKFWDAVKDYFAKFKE

SEQ ID NO: 280 - protein, 18 aa, Artificial Sequence
  synthetic construct; Class A amphipathic helical peptides
AFEKFKEAVKDYFAKFWD

SEQ ID NO: 281 - protein, 18 aa, Artificial Sequence
  synthetic construct; Class A amphipathic helical peptides
AFDKFKDAVKEYFAKFWE

SEQ ID NO: 282 - protein, 18 aa, Artificial Sequence
  synthetic construct; Class A amphipathic helical peptides
AFDKFKEAVKDYFAKFWE

SEQ ID NO: 283 - protein, 18 aa, Artificial Sequence
  synthetic construct; Class A amphipathic helical peptides
AFEKFKDAVKEYFAKFWD

SEQ ID NO: 284 - protein, 18 aa, Artificial Sequence
  synthetic construct; Class A amphipathic helical peptides
AFEKFKDAVKDYFAKFWE

SEQ ID NO: 285 - protein, 18 aa, Artificial Sequence
  synthetic construct; Class A amphipathic helical peptides
VAEKFKEAFKDYFAKFWD

SEQ ID NO: 286 - protein, 18 aa, Artificial Sequence
  synthetic construct; Class A amphipathic helical peptides
VADKFKDAFKEYFAKFWE

SEQ ID NO: 287 - protein, 18 aa, Artificial Sequence
  synthetic construct; Class A amphipathic helical peptides
VADKFKEAFKDYFAKFWE

SEQ ID NO: 288 - protein, 18 aa, Artificial Sequence
  synthetic construct; Class A amphipathic helical peptides
VAEKFKDAFKEYFAKFWD

SEQ ID NO: 289 - protein, 18 aa, Artificial Sequence
  synthetic construct; Class A amphipathic helical peptides
VAEKFKDAFKDYFAKFWE

SEQ ID NO: 290 - protein, 18 aa, Artificial Sequence
  synthetic construct; Class A amphipathic helical peptides
YAEKFKEAVKDFFAKFWD

SEQ ID NO: 291 - protein, 18 aa, Artificial Sequence
  synthetic construct; Class A amphipathic helical peptides
YADKFKDAVKEFFAKFWE

SEQ ID NO: 292 - protein, 18 aa, Artificial Sequence
  synthetic construct; Class A amphipathic helical peptides
YADKFKEAVKDFFAKFWE

SEQ ID NO: 293 - protein, 18 aa, Artificial Sequence
  synthetic construct; Class A amphipathic helical peptides
YAEKFKDAVKEFFAKFWD

SEQ ID NO: 294 - protein, 18 aa, Artificial Sequence
  synthetic construct; Class A amphipathic helical peptides
YAEKFKDAVKDFFAKFWE

SEQ ID NO: 295 - protein, 18 aa, Artificial Sequence
  synthetic construct; Class A amphipathic helical peptides
AAEKFKEFVKDYFAKFWD

SEQ ID NO: 296 - protein, 18 aa, Artificial Sequence
  synthetic construct; Class A amphipathic helical peptides
AADKFKDFVKEYFAKFWE

SEQ ID NO: 297 - protein, 18 aa, Artificial Sequence
  synthetic construct; Class A amphipathic helical peptides
AADKFKEFVKDYFAKFWE

SEQ ID NO: 298 - protein, 18 aa, Artificial Sequence
  synthetic construct; Class A amphipathic helical peptides
AAEKFKDFVKEYFAKFWD

SEQ ID NO: 299 - protein, 18 aa, Artificial Sequence
  synthetic construct; Class A amphipathic helical peptides
AAEKFKDFVKDYFAKFWE

SEQ ID NO: 300 - protein, 18 aa, Artificial Sequence
  synthetic construct; Class A amphipathic helical peptides
FFEKAKEAVKDYFAKFWD

SEQ ID NO: 301 - protein, 18 aa, Artificial Sequence
  synthetic construct; Class A amphipathic helical peptides
FFDKAKDAVKEYFAKFWE

SEQ ID NO: 302 - protein, 18 aa, Artificial Sequence
  synthetic construct; Class A amphipathic helical peptides
FFDKAKEAVKDYFAKFWE

SEQ ID NO: 303 - protein, 16 aa, Artificial Sequence
  synthetic construct; Class A amphipathic helical peptides
EKAKDAVKEYFAKFWD

SEQ ID NO: 304 - protein, 16 aa, Artificial Sequence
  synthetic construct; Class A amphipathic helical peptides
EKAKDAVKDYFAKFWE

SEQ ID NO: 305 - protein, 18 aa, Artificial Sequence
  synthetic construct; Class A amphipathic helical peptides
FYEKFKEAVKDAFAKFWD

SEQ ID NO: 306 - protein, 18 aa, Artificial Sequence
  synthetic construct; Class A amphipathic helical peptides
FYDKFKDAVKEAFAKFWE

SEQ ID NO: 307 - protein, 18 aa, Artificial Sequence
  synthetic construct; Class A amphipathic helical peptides
FYDKFKEAVKDAFAKFWE

SEQ ID NO: 308 - protein, 18 aa, Artificial Sequence
  synthetic construct; Class A amphipathic helical peptides
FYEKFKDAVKEAFAKFWD

SEQ ID NO: 309 - protein, 18 aa, Artificial Sequence
  synthetic construct; Class A amphipathic helical peptides
FYEKFKDAVKDAFAKFWE

SEQ ID NO: 310 - protein, 18 aa, Artificial Sequence
  synthetic construct; Class A amphipathic helical peptides
FVEKFKEAAKDYFAKFWD

SEQ ID NO: 311 - protein, 18 aa, Artificial Sequence
  synthetic construct; Class A amphipathic helical peptides
FVDKFKDAAKEYFAKFWE

SEQ ID NO: 312 - protein, 18 aa, Artificial Sequence
  synthetic construct; Class A amphipathic helical peptides
FVDKFKEAAKDYFAKFWE

SEQ ID NO: 313 - protein, 18 aa, Artificial Sequence
  synthetic construct; Class A amphipathic helical peptides
FVEKFKDAAKEYFAKFWD

SEQ ID NO: 314 - protein, 18 aa, Artificial Sequence
  synthetic construct; Class A amphipathic helical peptides
FVEKFKDAAKDYFAKFWE

SEQ ID NO: 315 - protein, 18 aa, Artificial Sequence
  synthetic construct; Class A amphipathic helical peptides
FAEKYKEAVKDFFAKFWD

SEQ ID NO: 316 - protein, 18 aa, Artificial Sequence
  synthetic construct; Class A amphipathic helical peptides
FADKYKDAVKEFFAKFWE

SEQ ID NO: 317 - protein, 18 aa, Artificial Sequence
  synthetic construct; Class A amphipathic helical peptides
FADKYKEAVKDFFAKFWE

SEQ ID NO: 318 - protein, 18 aa, Artificial Sequence
  synthetic construct; Class A amphipathic helical peptides
FAEKYKDAVKEFFAKFWD

SEQ ID NO: 319 - protein, 18 aa, Artificial Sequence
  synthetic construct; Class A amphipathic helical peptides
FAEKYKDAVKDFFAKFWE

SEQ ID NO: 320 - protein, 18 aa, Artificial Sequence
  synthetic construct; Class A amphipathic helical peptides
FAEKVKEAFKDYFAKFWD

SEQ ID NO: 321 - protein, 18 aa, Artificial Sequence
  synthetic construct; Class A amphipathic helical peptides
FADKVKDAFKEYFAKFWE

SEQ ID NO: 322 - protein, 18 aa, Artificial Sequence
  synthetic construct; Class A amphipathic helical peptides
FADKVKEAFKDYFAKFWE

SEQ ID NO: 323 - protein, 18 aa, Artificial Sequence
  synthetic construct; Class A amphipathic helical peptides
FAEKVKDAFKEYFAKFWD

SEQ ID NO: 324 - protein, 18 aa, Artificial Sequence
  synthetic construct; Class A amphipathic helical peptides
FAEKVKDAFKDYFAKFWE

SEQ ID NO: 325 - protein, 18 aa, Artificial Sequence
  synthetic construct; Class A amphipathic helical peptides
FAEKFKEYVKDAFAKFWD

SEQ ID NO: 326 - protein, 18 aa, Artificial Sequence
  synthetic construct; Class A amphipathic helical peptides
FADKFKDYVKEAFAKFWE

SEQ ID NO: 327 - protein, 18 aa, Artificial Sequence
  synthetic construct; Class A amphipathic helical peptides
FADKFKEYVKDAFAKFWE

SEQ ID NO: 328 - protein, 18 aa, Artificial Sequence
  synthetic construct; Class A amphipathic helical peptides
FAEKFKDYVKEAFAKFWD

SEQ ID NO: 329 - protein, 18 aa, Artificial Sequence
  synthetic construct; Class A amphipathic helical peptides
FAEKFKDYVKDAFAKFWE

SEQ ID NO: 330 - protein, 18 aa, Artificial Sequence
  synthetic construct; Class A amphipathic helical peptides
FAEKFKEAFKDYVAKFWD

SEQ ID NO: 331 - protein, 18 aa, Artificial Sequence
  synthetic construct; Class A amphipathic helical peptides
FADKFKDAFKEYVAKFWE

SEQ ID NO: 332 - protein, 18 aa, Artificial Sequence
  synthetic construct; Class A amphipathic helical peptides
FADKFKEAFKDYVAKFWE

SEQ ID NO: 333 - protein, 18 aa, Artificial Sequence
  synthetic construct; Class A amphipathic helical peptides
FAEKFKDAFKEYVAKFWD

SEQ ID NO: 334 - protein, 18 aa, Artificial Sequence
  synthetic construct; Class A amphipathic helical peptides
FAEKFKDAFKDYVAKFWE

SEQ ID NO: 335 - protein, 18 aa, Artificial Sequence
  synthetic construct; Class A amphipathic helical peptides
FAEKFKEAFKDYFAKVWD

SEQ ID NO: 336 - protein, 18 aa, Artificial Sequence
  synthetic construct; Class A amphipathic helical peptides
FADKFKDAFKEYFAKVWE

SEQ ID NO: 337 - protein, 18 aa, Artificial Sequence
  synthetic construct; Class A amphipathic helical peptides
FADKFKEAFKDYFAKVWE

SEQ ID NO: 338 - protein, 18 aa, Artificial Sequence
  synthetic construct; Class A amphipathic helical peptides
FAEKFKDAFKEYFAKVWD

SEQ ID NO: 339 - protein, 18 aa, Artificial Sequence
  synthetic construct; Class A amphipathic helical peptides
FAEKFKDAFKDYFAKVWE

SEQ ID NO: 340 - protein, 18 aa, Artificial Sequence
  synthetic construct; Class A amphipathic helical peptides
FAEKFKEAVKDFFAKYWD

SEQ ID NO: 341 - protein, 18 aa, Artificial Sequence
  synthetic construct; Class A amphipathic helical peptides
FADKFKDAVKEFFAKYWE

SEQ ID NO: 342 - protein, 18 aa, Artificial Sequence
  synthetic construct; Class A amphipathic helical peptides
FADKFKEAVKDFFAKYWE

SEQ ID NO: 343 - protein, 18 aa, Artificial Sequence
  synthetic construct; Class A amphipathic helical peptides
FAEKFKDAVKEFFAKYWD

SEQ ID NO: 344 - protein, 18 aa, Artificial Sequence
  synthetic construct; Class A amphipathic helical peptides
FAEKFKDAVKDFFAKYWE

SEQ ID NO: 345 - protein, 18 aa, Artificial Sequence
  synthetic construct; Class A amphipathic helical peptides
WAEKFFEAVKDYFAKFKD

SEQ ID NO: 346 - protein, 18 aa, Artificial Sequence
  synthetic construct; Class A amphipathic helical peptides
WADKFFDAVKEYFAKFKE

SEQ ID NO: 347 - protein, 18 aa, Artificial Sequence
  synthetic construct; Class A amphipathic helical peptides
WADKFFEAVKDYFAKFKE

SEQ ID NO: 348 - protein, 18 aa, Artificial Sequence
  synthetic construct; Class A amphipathic helical peptides
WAEKFFDAVKEYFAKFKD

SEQ ID NO: 349 - protein, 18 aa, Artificial Sequence
  synthetic construct; Class A amphipathic helical peptides
WAEKFFDAVKDYFAKFKE

SEQ ID NO: 350 - protein, 18 aa, Artificial Sequence
  synthetic construct; Class A amphipathic helical peptides
FAEKWFEAVKDYFAKFKD

SEQ ID NO: 351 - protein, 18 aa, Artificial Sequence
  synthetic construct; Class A amphipathic helical peptides
FADKWFDAVKEYFAKFKE

SEQ ID NO: 352 - protein, 18 aa, Artificial Sequence
  synthetic construct; Class A amphipathic helical peptides
FADKWFEAVKDYFAKFKE

SEQ ID NO: 353 - protein, 18 aa, Artificial Sequence
  synthetic construct; Class A amphipathic helical peptides
FAEKWFDAVKEYFAKFKD

SEQ ID NO: 354 - protein, 18 aa, Artificial Sequence
  synthetic construct; Class A amphipathic helical peptides
FAEKWFDAVKDYFAKFKE

SEQ ID NO: 355 - protein, 18 aa, Artificial Sequence
  synthetic construct; Class A amphipathic helical peptides
FAEKFVEAWKDYFAKFKD

SEQ ID NO: 356 - protein, 18 aa, Artificial Sequence
  synthetic construct; Class A amphipathic helical peptides
FADKFVDAWKEYFAKFKE

SEQ ID NO: 357 - protein, 18 aa, Artificial Sequence
  synthetic construct; Class A amphipathic helical peptides
FADKFVEAWKDYFAKFKE

SEQ ID NO: 358 - protein, 18 aa, Artificial Sequence
  synthetic construct; Class A amphipathic helical peptides
FAEKFVDAWKEYFAKFKD

SEQ ID NO: 359 - protein, 18 aa, Artificial Sequence
  synthetic construct; Class A amphipathic helical peptides
FAEKFVDAWKDYFAKFKE

SEQ ID NO: 360 - protein, 18 aa, Artificial Sequence
  synthetic construct; Class A amphipathic helical peptides
FYEKFAEAVKDWFAKFKD

SEQ ID NO: 361 - protein, 18 aa, Artificial Sequence
  synthetic construct; Class A amphipathic helical peptides
FYDKFADAVKEWFAKFKE

SEQ ID NO: 362 - protein, 18 aa, Artificial Sequence
  synthetic construct; Class A amphipathic helical peptides
FYDKFAEAVKDWFAKFKE

SEQ ID NO: 363 - protein, 18 aa, Artificial Sequence
  synthetic construct; Class A amphipathic helical peptides
FYEKFADAVKEWFAKFKD

SEQ ID NO: 364 - protein, 18 aa, Artificial Sequence
  synthetic construct; Class A amphipathic helical peptides
FYEKFADAVKDWFAKFKE

SEQ ID NO: 365 - protein, 18 aa, Artificial Sequence
  synthetic construct; class A or class Y amphipathic helix peptide
  misc (1)..(1): D can be Asp or Glu
  misc (2)..(3): Xaa can be Leu, norLeu, Val, Ile, Trp, Phe, Tyr, beta-Nal, or alpha-Nal
  misc (5)..(5): Y can be Ala, His, Ser, Gln, Asn, or Thr
  misc (6)..(7): Xaa can be Leu, norLeu, Val, Ile, Trp, Phe, Tyr, beta-Nal, or alpha-Nal
  misc (8)..(8): D can be Asp or Glu
  misc (10)..(10): Xaa can be Leu, norLeu, Val, Ile, Trp, Phe, Tyr, beta-Nal, or alpha-Nal
  misc (11)..(11): Y can be Ala, His, Ser, Gln, Asn, or Thr
  misc (12)..(12): D can be Asp or Glu
  misc (14)..(14): Xaa can be Leu, norLeu, Val, Ile, Trp, Phe, Tyr, beta-Nal, or alpha-Nal
  misc (16)..(16): D can be Asp or Glu
  misc (17)..(17): Y can be Ala, His, Ser, Gln, Asn, or Thr
  misc (18)..(18): Xaa can be Leu, norLeu, Val, Ile, Trp, Phe, Tyr, beta-Nal, or alpha-Nal
DXXKYXXDKXYDKXKDYX

SEQ ID NO: 366 - protein, 18 aa, Artificial Sequence
  synthetic construct; peptide mimetic
DWFKHFYDKVAEKFKEAF

SEQ ID NO: 367 - protein, 18 aa, Artificial Sequence
  synthetic construct; peptide mimetic
EWFKHFYEKVADKFKDAF

SEQ ID NO: 368 - protein, 18 aa, Artificial Sequence
  synthetic construct; peptide mimetic
EWFKHFYDKVAEKFKEAF

SEQ ID NO: 369 - protein, 18 aa, Artificial Sequence
  synthetic construct; peptide mimetic
DWFKHFYEKVAEKFKEAF

SEQ ID NO: 370 - protein, 18 aa, Artificial Sequence
  synthetic construct; peptide mimetic
DWFKHFYDKVADKFKEAF

SEQ ID NO: 371 - protein, 18 aa, Artificial Sequence
  synthetic construct; peptide mimetic
DWFKHFYDKVAEKFKDAF

SEQ ID NO: 372 - protein, 18 aa, Artificial Sequence
  synthetic construct; peptide mimetic
DWHKFFYDKVAEKFKEAF

SEQ ID NO: 373 - protein, 18 aa, Artificial Sequence
  synthetic construct; peptide mimetic
EWHKFFYEKVADKFKDAF

SEQ ID NO: 374 - protein, 18 aa, Artificial Sequence
  synthetic construct; peptide mimetic
EWHKFFYDKVAEKFKEAF

SEQ ID NO: 375 - protein, 18 aa, Artificial Sequence
  synthetic construct; peptide mimetic
DWHKFFYEKVAEKFKEAF

SEQ ID NO: 376 - protein, 18 aa, Artificial Sequence
  synthetic construct; peptide mimetic
DWHKFFYDKVADKFKEAF

SEQ ID NO: 377 - protein, 18 aa, Artificial Sequence
  synthetic construct; peptide mimetic
DWHKFFYDKVAEKFKDAF

SEQ ID NO: 378 - protein, 18 aa, Artificial Sequence
  synthetic construct; peptide mimetic
DWFKFHYDKVAEKFKEAF

SEQ ID NO: 379 - protein, 18 aa, Artificial Sequence
  synthetic construct; peptide mimetic
EWFKFHYEKVADKFKDAF

SEQ ID NO: 380 - protein, 18 aa, Artificial Sequence
  synthetic construct; peptide mimetic
EWFKFHYDKVAEKFKEAF

SEQ ID NO: 381 - protein, 18 aa, Artificial Sequence
  synthetic construct; peptide mimetic
DWFKFHYEKVAEKFKEAF

SEQ ID NO: 382 - protein, 18 aa, Artificial Sequence
  synthetic construct; peptide mimetic
DWFKFHYDKVADKFKEAF

SEQ ID NO: 383 - protein, 18 aa, Artificial Sequence
  synthetic construct; peptide mimetic
DWFKFHYDKVAEKFKDAF

SEQ ID NO: 384 - protein, 18 aa, Artificial Sequence
  synthetic construct; peptide mimetic
DWFKVFYDKHAEKFKEAF

SEQ ID NO: 385 - protein, 18 aa, Artificial Sequence
  synthetic construct; peptide mimetic
EWFKVFYEKHADKFKDAF

SEQ ID NO: 386 - protein, 18 aa, Artificial Sequence
  synthetic construct; peptide mimetic
EWFKVFYDKHAEKFKEAF

SEQ ID NO: 387 - protein, 18 aa, Artificial Sequence
  synthetic construct; peptide mimetic
DWFKVFYEKHAEKFKEAF

SEQ ID NO: 388 - protein, 18 aa, Artificial Sequence
  synthetic construct; peptide mimetic
DWFKVFYDKHADKFKEAF

SEQ ID NO: 389 - protein, 18 aa, Artificial Sequence
  synthetic construct; peptide mimetic
DWFKVFYDKHAEKFKDAF

SEQ ID NO: 390 - protein, 18 aa, Artificial Sequence
  synthetic construct; peptide mimetic
DWFKAFYDKVAEKFKEHF

SEQ ID NO: 391 - protein, 18 aa, Artificial Sequence
  synthetic construct; peptide mimetic
EWFKAFYEKVADKFKDHF

SEQ ID NO: 392 - protein, 18 aa, Artificial Sequence
  synthetic construct; peptide mimetic
EWFKAFYDKVAEKFKEHF

SEQ ID NO: 393 - protein, 18 aa, Artificial Sequence
  synthetic construct; peptide mimetic
DWFKAFYEKVAEKFKEHF

SEQ ID NO: 394 - protein, 18 aa, Artificial Sequence
  synthetic construct; peptide mimetic
DWFKAFYDKVADKFKEHF

SEQ ID NO: 395 - protein, 18 aa, Artificial Sequence
  synthetic construct; peptide mimetic
DWFKAFYDKVAEKFKDHF

SEQ ID NO: 396 - protein, 18 aa, Artificial Sequence
  synthetic construct; peptide mimetic
DWFKAFYDKVAEKFKEFH

SEQ ID NO: 397 - protein, 18 aa, Artificial Sequence
  synthetic construct; peptide mimetic
EWFKAFYEKVADKFKDFH

SEQ ID NO: 398 - protein, 18 aa, Artificial Sequence
  synthetic construct; peptide mimetic
EWFKAFYDKVAEKFKEFH

SEQ ID NO: 399 - protein, 18 aa, Artificial Sequence
  synthetic construct; peptide mimetic
DWFKAFYDKVAEKFKEFH

SEQ ID NO: 400 - protein, 18 aa, Artificial Sequence
  synthetic construct; peptide mimetic
DWFKAFYEKVAEKFKEFH

SEQ ID NO: 401 - protein, 18 aa, Artificial Sequence
  synthetic construct; peptide mimetic
DWFKAFYDKVAEKFKEFH

SEQ ID NO: 402 - protein, 18 aa, Artificial Sequence
  synthetic construct; peptide mimetic
DWFKAFYDKVAEKFKDFH

SEQ ID NO: 403 - protein, 18 aa, Artificial Sequence
  synthetic construct; peptide mimetic
FAEKFKEAVKDYFAKFWD

SEQ ID NO: 404 - protein, 18 aa, Artificial Sequence
  synthetic construct; peptide mimetic
FHEKFKEAVKDYFAKFWD

SEQ ID NO: 405 - protein, 18 aa, Artificial Sequence
  synthetic construct; peptide mimetic
FHEKFKEAVKEYFAKFWE

SEQ ID NO: 406 - protein, 18 aa, Artificial Sequence
  synthetic construct; peptide mimetic
FHDKFKDAVKDYFAKFWD

SEQ ID NO: 407 - protein, 18 aa, Artificial Sequence
  synthetic construct; peptide mimetic
FHDKFKDAVKEYFAKFWE

SEQ ID NO: 408 - protein, 18 aa, Artificial Sequence
  synthetic construct; peptide mimetic
FHDKFKEAVKDYFAKFWD

SEQ ID NO: 409 - protein, 18 aa, Artificial Sequence
  synthetic construct; peptide mimetic
FHEKFKDAVKDYFAKFWD

SEQ ID NO: 410 - protein, 18 aa, Artificial Sequence
  synthetic construct; peptide mimetic
FHEKFKEAVKEYFAKFWD

SEQ ID NO: 411 - protein, 18 aa, Artificial Sequence
  synthetic construct; peptide mimetic
FHEKFKEAVKDYFAKFWE

SEQ ID NO: 412 - protein, 18 aa, Artificial Sequence
  synthetic construct; peptide mimetic
HFEKFKEAVKDYFAKFWD

SEQ ID NO: 413 - protein, 18 aa, Artificial Sequence
  synthetic construct; peptide mimetic
HFDKFKDAVKEYFAKFWE

SEQ ID NO: 414 - protein, 18 aa, Artificial Sequence
  synthetic construct; peptide mimetic
HFEKFKEAVKEYFAKFWE

SEQ ID NO: 415 - protein, 18 aa, Artificial Sequence
  synthetic construct; peptide mimetic
HFDKFKEAVKDYFAKFWD

SEQ ID NO: 416 - protein, 18 aa, Artificial Sequence
  synthetic construct; peptide mimetic
HFEKFKDAVKDYFAKFWD

SEQ ID NO: 417 - protein, 18 aa, Artificial Sequence
  synthetic construct; peptide mimetic
HFEKFKEAVKEYFAKFWD

SEQ ID NO: 418 - protein, 18 aa, Artificial Sequence
  synthetic construct; peptide mimetic
HFEKFKEAVKDYFAKFWE

SEQ ID NO: 419 - protein, 18 aa, Artificial Sequence
  synthetic construct; peptide mimetic
FFEKHKEAVKDYFAKFWD

SEQ ID NO: 420 - protein, 18 aa, Artificial Sequence
  synthetic construct; peptide mimetic
FFDKHKDAVKEYFAKFWE

SEQ ID NO: 421 - protein, 18 aa, Artificial Sequence
  synthetic construct; peptide mimetic
FFEKHKEAVKEYFAKFWE

SEQ ID NO: 422 - protein, 18 aa, Artificial Sequence
  synthetic construct; peptide mimetic
FFDKHKDAVKDYFAKFWD

SEQ ID NO: 423 - protein, 18 aa, Artificial Sequence
  synthetic construct; peptide mimetic
FFDKHKEAVKDYFAKFWD

SEQ ID NO: 424 - protein, 18 aa, Artificial Sequence
  synthetic construct; peptide mimetic
FFEKHKEAVKEYFAKFWD

SEQ ID NO: 425 - protein, 18 aa, Artificial Sequence
  synthetic construct; peptide mimetic
FFEKHKEAVKDYFAKFWE

SEQ ID NO: 426 - protein, 18 aa, Artificial Sequence
  synthetic construct; peptide mimetic
FVEKFKEAHKDYFAKFWD

SEQ ID NO: 427 - protein, 18 aa, Artificial Sequence
  synthetic construct; peptide mimetic
FVDKFKDAHKEYFAKFWE

SEQ ID NO: 428 - protein, 18 aa, Artificial Sequence
  synthetic construct; peptide mimetic
FVEKFKEAHKEYFAKFWE

SEQ ID NO: 429 - protein, 18 aa, Artificial Sequence
  synthetic construct; peptide mimetic
FVDKFKDAHKDYFAKFWD

SEQ ID NO: 430 - protein, 18 aa, Artificial Sequence
  synthetic construct; peptide mimetic
FVDKFKEAHKDYFAKFWD

SEQ ID NO: 431 - protein, 18 aa, Artificial Sequence
  synthetic construct; peptide mimetic
FVEKFKDAHKDYFAKFWD

SEQ ID NO: 432 - protein, 18 aa, Artificial Sequence
  synthetic construct; peptide mimetic
FVEKFKEAHKEYFAKFWD

SEQ ID NO: 433 - protein, 18 aa, Artificial Sequence
  synthetic construct; peptide mimetic
FVEKFKEAHKDYFAKFWE

SEQ ID NO: 434 - protein, 18 aa, Artificial Sequence
  synthetic construct; peptide mimetic
FAEKFKEHVKDYFAKFWD

SEQ ID NO: 435 - protein, 18 aa, Artificial Sequence
  synthetic construct; peptide mimetic
FADKFKDHVKEYFAKFWE

SEQ ID NO: 436 - protein, 18 aa, Artificial Sequence
  synthetic construct; peptide mimetic
FAEKFKEHVKEYFAKFWE

SEQ ID NO: 437 - protein, 18 aa, Artificial Sequence
  synthetic construct; peptide mimetic
FADKFKDHVKDYFAKFWD

SEQ ID NO: 438 - protein, 18 aa, Artificial Sequence
  synthetic construct; peptide mimetic
FADKFKEHVKDYFAKFWD

SEQ ID NO: 439 - protein, 18 aa, Artificial Sequence
  synthetic construct; peptide mimetic
FAEKFKDHVKDYFAKFWD

SEQ ID NO: 440 - protein, 18 aa, Artificial Sequence
  synthetic construct; peptide mimetic
FAEKFKEHVKEYFAKFWD

SEQ ID NO: 441 - protein, 18 aa, Artificial Sequence
  synthetic construct; peptide mimetic
FAEKFKEHVKDYFAKFWE

SEQ ID NO: 442 - protein, 18 aa, Artificial Sequence
  synthetic construct; peptide mimetic
FAEKFKEFVKDYHAKFWD

SEQ ID NO: 443 - protein, 18 aa, Artificial Sequence
  synthetic construct; peptide mimetic
FADKFKDFVKEYHAKFWE

SEQ ID NO: 444 - protein, 18 aa, Artificial Sequence
  synthetic construct; peptide mimetic
FADKFKEFVKDYHAKFWD

SEQ ID NO: 445 - protein, 18 aa, Artificial Sequence
  synthetic construct; peptide mimetic
FAEKFKDFVKDYHAKFWD

SEQ ID NO: 446 - protein, 18 aa, Artificial Sequence
  synthetic construct; peptide mimetic
FADKFKDFVKDYHAKFWD

SEQ ID NO: 447 - protein, 18 aa, Artificial Sequence
  synthetic construct; peptide mimetic
FAEKFKEFVKEYHAKFWE

SEQ ID NO: 448 - protein, 18 aa, Artificial Sequence
  synthetic construct; peptide mimetic
FAEKFKEFVKEYHAKFWD

SEQ ID NO: 449 - protein, 18 aa, Artificial Sequence
  synthetic construct; peptide mimetic
FAEKFKEFVKDYHAKFWE

SEQ ID NO: 450 - protein, 18 aa, Artificial Sequence
  synthetic construct; peptide mimetic
FAEKFKEFVKDYFAKHWD

SEQ ID NO: 451 - protein, 18 aa, Artificial Sequence
  synthetic construct; peptide mimetic
FADKFKDFVKEYFAKHWE

SEQ ID NO: 452 - protein, 18 aa, Artificial Sequence
  synthetic construct; peptide mimetic
FAEKFKEFVKEYFAKHWE

SEQ ID NO: 453 - protein, 18 aa, Artificial Sequence
  synthetic construct; peptide mimetic
FADKFKDFVKDYFAKHWD

SEQ ID NO: 454 - protein, 18 aa, Artificial Sequence
  synthetic construct; peptide mimetic
FADKFKEFVKDYFAKHWD

SEQ ID NO: 455 - protein, 18 aa, Artificial Sequence
  synthetic construct; peptide mimetic
FAEKFKDFVKDYFAKHWD

SEQ ID NO: 456 - protein, 18 aa, Artificial Sequence
  synthetic construct; peptide mimetic
FAEKFKEFVKEYFAKHWD

SEQ ID NO: 457 - protein, 18 aa, Artificial Sequence
  synthetic construct; peptide mimetic
FAEKFKEFVKDYFAKHWE

SEQ ID NO: 458 - protein, 18 aa, Artificial Sequence
  synthetic construct, Nph peptide mimetic
  misc (3)..(3): The phenyl group comprises a para nitro moiety
  misc (6)..(6): The phenyl group comprises a para nitro moiety
  misc (14)..(14): The phenyl group comprises a para nitro moiety
  misc (18)..(18): The phenyl group comprises a para nitro moiety
DWFKAFYDKVAEKFKEAF

SEQ ID NO: 459 - protein, 18 aa, Artificial Sequence
  synthetic construct, Nph peptide mimetic
  misc (3)..(3): The phenyl group comprises a para nitro moiety
  misc (6)..(6): The phenyl group comprises a para nitro moiety
  misc (14)..(14): The phenyl group comprises a para nitro moiety
  misc (18)..(18): The phenyl group comprises a para nitro moiety
EWFKAFYEKVADKFKDAF

SEQ ID NO: 460 - protein, 18 aa, Artificial Sequence
  synthetic construct, Nph peptide mimetic
  misc (3)..(3): The phenyl group comprises a para nitro moiety
  misc (6)..(6): The phenyl group comprises a para nitro moiety
  misc (14)..(14): The phenyl group comprises a para nitro moiety
  misc (18)..(18): The phenyl group comprises a para nitro moiety
EWFKAFYEKVAEKFKEAF

SEQ ID NO: 461 - protein, 18 aa, Artificial Sequence
  synthetic construct, Nph peptide mimetic
  misc (3)..(3): The phenyl group comprises a para nitro moiety
  misc (6)..(6): The phenyl group comprises a para nitro moiety
  misc (14)..(14): The phenyl group comprises a para nitro moiety
  misc (18)..(18): The phenyl group comprises a para nitro moiety
DWFKAFYDKVADKFKDAF

SEQ ID NO: 462 - protein, 18 aa, Artificial Sequence
  synthetic construct, Nph peptide mimetic
  misc (3)..(3): The phenyl group comprises a para nitro moiety
  misc (6)..(6): The phenyl group comprises a para nitro moiety
  misc (14)..(14): The phenyl group comprises a para nitro moiety
  misc (18)..(18): The phenyl group comprises a para nitro moiety
EWFKAFYDKVAEKFKEAF

SEQ ID NO: 463 - protein, 18 aa, Artificial Sequence
  synthetic construct, Nph peptide mimetic
  misc (3)..(3): The phenyl group comprises a para nitro moiety
  misc (6)..(6): The phenyl group comprises a para nitro moiety
  misc (14)..(14): The phenyl group comprises a para nitro moiety
  misc (18)..(18): The phenyl group comprises a para nitro moiety
DWFKAFYEKVAEKFKEAF

SEQ ID NO: 464 - protein, 18 aa, Artificial Sequence
  synthetic construct, Nph peptide mimetic
  misc (3)..(3): The phenyl group comprises a para nitro moiety
  misc (6)..(6): The phenyl group comprises a para nitro moiety
  misc (14)..(14): The phenyl group comprises a para nitro moiety
  misc (18)..(18): The phenyl group comprises a para nitro moiety
DWFKAFYDKVADKFKEAF

SEQ ID NO: 465 - protein, 18 aa, Artificial Sequence
  synthetic construct, Nph peptide mimetic
  misc (3)..(3): The phenyl group comprises a para nitro moiety
  misc (6)..(6): The phenyl group comprises a para nitro moiety
  misc (14)..(14): The phenyl group comprises a para nitro moiety
  misc (18)..(18): The phenyl group comprises a para nitro moiety
DWFKAFYDKVAEKFKDAF

SEQ ID NO: 466 - protein, 18 aa, Artificial Sequence
  synthetic construct, Nph peptide mimetic
  misc (3)..(3): The phenyl group comprises a para nitro moiety
  misc (6)..(6): The phenyl group comprises a para nitro moiety
  misc (14)..(14): The phenyl group comprises a para nitro moiety
  misc (18)..(18): The phenyl group comprises a para nitro moiety
DWFKAFYDKVAEKFKEAF

SEQ ID NO: 467 - protein, 18 aa, Artificial Sequence
  synthetic construct, Nph peptide mimetic
  misc (3)..(3): The phenyl group comprises a para nitro moiety
  misc (6)..(6): The phenyl group comprises a para nitro moiety
  misc (14)..(14): The phenyl group comprises a para nitro moiety
  misc (18)..(18): The phenyl group comprises a para nitro moiety
DWFKAFYDKVAEKFKEAF

SEQ ID NO: 468 - protein, 18 aa, Artificial Sequence
  synthetic construct, Nph peptide mimetic
  misc (3)..(3): The phenyl group comprises a para nitro moiety
  misc (6)..(6): The phenyl group comprises a para nitro moiety
  misc (14)..(14): The phenyl group comprises a para nitro moiety
  misc (18)..(18): The phenyl group comprises a para nitro moiety
DWFKAFYDKVAEKFKEAF

SEQ ID NO: 469 - protein, 18 aa, Artificial Sequence
  synthetic construct, Nph peptide mimetic
  misc (3)..(3): The phenyl group comprises a para nitro moiety
  misc (6)..(6): The phenyl group comprises a para nitro moiety
  misc (14)..(14): The phenyl group comprises a para nitro moiety
  misc (18)..(18): The phenyl group comprises a para nitro moiety
DWFKAFYDKVAEKFKEAF

SEQ ID NO: 470 - protein, 18 aa, Artificial Sequence
  synthetic construct, Nph peptide mimetic
  misc (3)..(3): The phenyl group comprises a para nitro moiety
  misc (6)..(6): The phenyl group comprises a para nitro moiety
  misc (14)..(14): The phenyl group comprises a para nitro moiety
  misc (18)..(18): The phenyl group comprises a para nitro moiety
DWFKAFYDKVAEKFKEAF

SEQ ID NO: 471 - protein, 18 aa, Artificial Sequence
  synthetic construct, Nph peptide mimetic
  misc (3)..(3): The phenyl group comprises a para nitro moiety
  misc (6)..(6): The phenyl group comprises a para nitro moiety
  misc (14)..(14): The phenyl group comprises a para nitro moiety
  misc (18)..(18): The phenyl group comprises a para nitro moiety
DWFKAFYDKVAEKFKEAF

SEQ ID NO: 472 - protein, 18 aa, Artificial Sequence
  synthetic construct, Nph peptide mimetic
  misc (1)..(1): The phenyl group comprises a para nitro moiety
  misc (5)..(5): The phenyl group comprises a para nitro moiety
  misc (13)..(13): The phenyl group comprises a para nitro moiety
  misc (16)..(16): The phenyl group comprises a para nitro moiety
FAEKFKEAVKDYFAKFWD

SEQ ID NO: 473 - protein, 18 aa, Artificial Sequence
  synthetic construct, Nph peptide mimetic
  misc (1)..(1): The phenyl group comprises a para nitro moiety
  misc (5)..(5): The phenyl group comprises a para nitro moiety
FAEKFKEAVKDYFAKFWD

SEQ ID NO: 474 - protein, 18 aa, Artificial Sequence
  synthetic construct, Nph peptide mimetic
  misc (13)..(13): The phenyl group comprises a para nitro moiety
  misc (16)..(16): The phenyl group comprises a para nitro moiety
FAEKFKEAVKDYFAKFWD

SEQ ID NO: 475 - protein, 18 aa, Artificial Sequence
  synthetic construct, Nph peptide mimetic
  misc (1)..(1): The phenyl group comprises a para nitro moiety
FAEKFKEAVKDYFAKFWD

SEQ ID NO: 476 - protein, 18 aa, Artificial Sequence
  synthetic construct, Nph peptide mimetic
  misc (5)..(5): The phenyl group comprises a para nitro moiety
FAEKFKEAVKDYFAKFWD

SEQ ID NO: 477 - protein, 18 aa, Artificial Sequence
  synthetic construct, Nph peptide mimetic
  misc (13)..(13): The phenyl group comprises a para nitro moiety
FAEKFKEAVKDYFAKFWD

SEQ ID NO: 478 - protein, 18 aa, Artificial Sequence
  synthetic construct, Nph peptide mimetic
  misc (16)..(16): The phenyl group comprises a para nitro moiety
FAEKEKEAVKDYFAKFWD

SEQ ID NO: 479 - protein, 18 aa, Artificial Sequence
  synthetic construct; peptide mimetic
FAEKFKEAVKEYFAKFWE

SEQ ID NO: 480 - protein, 18 aa, Artificial Sequence
  synthetic construct; peptide mimetic
FADKFKDAVKDYFAKFWD

SEQ ID NO: 481 - protein, 18 aa, Artificial Sequence
  synthetic construct; peptide mimetic
FAERFREAVKDYFAKFWD

SEQ ID NO: 482 - protein, 18 aa, Artificial Sequence
  synthetic construct; peptide mimetic
FAEKFREAVKDYFAKFWD

SEQ ID NO: 483 - protein, 18 aa, Artificial Sequence
  synthetic construct; peptide mimetic
FAEKFKEAVRDYFAKFWD

SEQ ID NO: 484 - protein, 18 aa, Artificial Sequence
  synthetic construct; peptide mimetic
FAEKFKEAVKDYFARFWD

SEQ ID NO: 485 - protein, 18 aa, Artificial Sequence
  synthetic construct; peptide mimetic
FAEKFREAVKDYEAKFWD

SEQ ID NO: 486 - protein, 18 aa, Artificial Sequence
  synthetic construct; peptide mimetic
LFEKFAEAFKDYVAKWKD

SEQ ID NO: 487 - protein, 18 aa, Artificial Sequence
  synthetic construct; peptide mimetic
LFERFAEAFKDYVAKWKD

SEQ ID NO: 488 - protein, 18 aa, Artificial Sequence
  synthetic construct; peptide mimetic
LFEKFAEAFRDYVAKWKD

SEQ ID NO: 489 - protein, 18 aa, Artificial Sequence
  synthetic construct; peptide mimetic
LFEKFAEAFKDYVARWKD

SEQ ID NO: 490 - protein, 18 aa, Artificial Sequence
  synthetic construct; peptide mimetic
LFEKFAEAFKDYVAKWRD

SEQ ID NO: 491 - protein, 18 aa, Artificial Sequence
  synthetic construct; peptide mimetic
LFEKFAEAFKEYVAKWKE

SEQ ID NO: 492 - protein, 18 aa, Artificial Sequence
  synthetic construct; peptide mimetic
LFDKFADAFKDYVAKWKD

SEQ ID NO: 493 - protein, 18 aa, Artificial Sequence
  synthetic construct; peptide mimetic
LFDKFAEAFKDYVAKWKD

SEQ ID NO: 494 - protein, 18 aa, Artificial Sequence
  synthetic construct; peptide mimetic
LFEKFADAFKDYVAKWKD

SEQ ID NO: 495 - protein, 18 aa, Artificial Sequence
  synthetic construct; peptide mimetic
LFEKFAEAFKEYVAKWKD

SEQ ID NO: 496 - protein, 18 aa, Artificial Sequence
  synthetic construct; peptide mimetic
LFEKFAEAFKDYVAKWKE

SEQ ID NO: 497 - protein, 18 aa, Artificial Sequence
  synthetic construct; peptide mimetic
FAEKAWEFVKDYFAKLKD

SEQ ID NO: 498 - protein, 18 aa, Artificial Sequence
  synthetic construct; peptide mimetic
FAERAWEFVKDYFAKLKD

SEQ ID NO: 499 - protein, 18 aa, Artificial Sequence
  synthetic construct; peptide mimetic
FAEKAWEFVKDYFAKLKD

SEQ ID NO: 500 - protein, 18 aa, Artificial Sequence
  synthetic construct; peptide mimetic
FAEKAWEFVKDYFAKLKD

SEQ ID NO: 501 - protein, 18 aa, Artificial Sequence
  synthetic construct; peptide mimetic
FAEKAWEFVKDYFAKLRD

SEQ ID NO: 502 - protein, 18 aa, Artificial Sequence
  synthetic construct; peptide mimetic
FAEKAWEFVKEYFAKLKE

SEQ ID NO: 503 - protein, 18 aa, Artificial Sequence
  synthetic construct; peptide mimetic
FADKAWDFVKDYFAKLKD

SEQ ID NO: 504 - protein, 18 aa, Artificial Sequence
  synthetic construct; peptide mimetic
FADKAWEFVKDYFAKLKD

SEQ ID NO: 505 - protein, 18 aa, Artificial Sequence
  synthetic construct; peptide mimetic
FAEKAWDFVKDYFAKLKD

SEQ ID NO: 506 - protein, 18 aa, Artificial Sequence
  synthetic construct; peptide mimetic
FAEKAWEFVKEYFAKLKD

SEQ ID NO: 507 - protein, 18 aa, Artificial Sequence
  synthetic construct; peptide mimetic
FAEKAWEFVKDYFAKLKE

SEQ ID NO: 508 - protein, 18 aa, Artificial Sequence
  synthetic construct; peptide mimetic
FFEKFKEFVKDYFAKLWD

SEQ ID NO: 509 - protein, 18 aa, Artificial Sequence
  synthetic construct; peptide mimetic
FFEKFKEFVKEYFAKLWE

SEQ ID NO: 510 - protein, 18 aa, Artificial Sequence
  synthetic construct; peptide mimetic
FFDKFKDFVKDYFAKLWD

SEQ ID NO: 511 - protein, 18 aa, Artificial Sequence
  synthetic construct; peptide mimetic
FFERFKEFVKDYFAKLWD

SEQ ID NO: 512 - protein, 18 aa, Artificial Sequence
  synthetic construct; peptide mimetic
FFEKFREFVKDYFAKLWD

SEQ ID NO: 513 - protein, 18 aa, Artificial Sequence
  synthetic construct; peptide mimetic
FFEKFKEFVRDYFAKLWD

SEQ ID NO: 514 - protein, 18 aa, Artificial Sequence
  synthetic construct; peptide mimetic
FFEKFKEFVKDYFARLWD

SEQ ID NO: 515 - protein, 18 aa, Artificial Sequence
  synthetic construct; peptide mimetic
FFDKFKEFVKDYFAKLWD

SEQ ID NO: 516 - protein, 18 aa, Artificial Sequence
  synthetic construct; peptide mimetic
FFEKFKDFVKDYFAKLWD

SEQ ID NO: 517 - protein, 18 aa, Artificial Sequence
  synthetic construct; peptide mimetic
FFEKFKEFVKEYFAKLWD

SEQ ID NO: 518 - protein, 18 aa, Artificial Sequence
  synthetic construct; peptide mimetic
FFEKFKEFVKDYFAKLWE

SEQ ID NO: 519 - protein, 18 aa, Artificial Sequence
  synthetic construct; peptide mimetic
FLEKFKEFVKDYFAKFWD

SEQ ID NO: 520 - protein, 18 aa, Artificial Sequence
  synthetic construct; peptide mimetic
FLEKFKEFVKEYFAKFWE

SEQ ID NO: 521 - protein, 18 aa, Artificial Sequence
  synthetic construct; peptide mimetic
FLDKFKEFVKDYFAKFWD

SEQ ID NO: 522 - protein, 18 aa, Artificial Sequence
  synthetic construct; peptide mimetic
FLDKFKEFVKDYFAKFWD

SEQ ID NO: 523 - protein, 18 aa, Artificial Sequence
  synthetic construct; peptide mimetic
FLEKFKDFVKDYFAKFWD

SEQ ID NO: 524 - protein, 18 aa, Artificial Sequence
  synthetic construct; peptide mimetic
FLEKFKEFVKEYFAKFWD

SEQ ID NO: 525 - protein, 18 aa, Artificial Sequence
  synthetic construct; peptide mimetic
FLEKFKEFVKDYFAKFWE

SEQ ID NO: 526 - protein, 18 aa, Artificial Sequence
  synthetic construct; peptide mimetic
FLERFKEFVKDYFAKFWD

SEQ ID NO: 527 - protein, 18 aa, Artificial Sequence
  synthetic construct; peptide mimetic
FLEKFREFVKDYFAKFWD

SEQ ID NO: 528 - protein, 18 aa, Artificial Sequence
  synthetic construct; peptide mimetic
FLEKFKEFVRDYFAKFWD

SEQ ID NO: 529 - protein, 18 aa, Artificial Sequence
  synthetic construct; peptide mimetic
FLEKFKEFVKDYFARFWD

SEQ ID NO: 530 - protein, 18 aa, Artificial Sequence
  synthetic construct; peptide mimetic
FFEKFKEFFKDYFAKLWD

SEQ ID NO: 531 - protein, 18 aa, Artificial Sequence
  synthetic construct; peptide mimetic
FFEKFKEFFKEYFAKLWE

SEQ ID NO: 532 - protein, 18 aa, Artificial Sequence
  synthetic construct; peptide mimetic
FFDKFKDFFKDYFAKLWD

SEQ ID NO: 533 - protein, 18 aa, Artificial Sequence
  synthetic construct; peptide mimetic
FFERFKEFFKDYFAKLWD

SEQ ID NO: 534 - protein, 18 aa, Artificial Sequence
  synthetic construct; peptide mimetic
FFEKFREFFKDYFAKLWD

SEQ ID NO: 535 - protein, 18 aa, Artificial Sequence
  synthetic construct; peptide mimetic
FFEKFKEFFRDYFAKLWD

SEQ ID NO: 536 - protein, 18 aa, Artificial Sequence
  synthetic construct; peptide mimetic
FFERFKEFFKDYFARLWD

SEQ ID NO: 537 - protein, 18 aa, Artificial Sequence
  synthetic construct; peptide mimetic
FFDKFKEFFKDYFAKLWD

SEQ ID NO: 538 - protein, 18 aa, Artificial Sequence
  synthetic construct; peptide mimetic
FFEKEKDFFKDYFAKLWD

SEQ ID NO: 539 - protein, 18 aa, Artificial Sequence
  synthetic construct; peptide mimetic
FFEKFKEFFKEYFAKLWD

SEQ ID NO: 540 - protein, 18 aa, Artificial Sequence
  synthetic construct; peptide mimetic
FFEKFKEFFKDYFAKLWE

SEQ ID NO: 541 - protein, 18 aa, Artificial Sequence
  synthetic construct; peptide mimetic
FAEKFKEAVKDYFAKFWD

SEQ ID NO: 542 - protein, 18 aa, Artificial Sequence
  synthetic construct; peptide mimetic
DKWKAVYDKFAEAFKEFF

SEQ ID NO: 543 - protein, 18 aa, Artificial Sequence
  synthetic construct; peptide mimetic
EKWKAVYEKFAEAFKEFF

SEQ ID NO: 544 - protein, 18 aa, Artificial Sequence
  synthetic construct; peptide mimetic
DKWKAVYDKFADAFKDFF

SEQ ID NO: 545 - protein, 18 aa, Artificial Sequence
  synthetic construct; peptide mimetic
DRWKAVYDKFAEAFKEFF

SEQ ID NO: 546 - protein, 18 aa, Artificial Sequence
  synthetic construct; peptide mimetic
DKWRAVYDKFAEAFKEFF

SEQ ID NO: 547 - protein, 18 aa, Artificial Sequence
  synthetic construct; peptide mimetic
DKWKAVYDRFAEAFKEFF

SEQ ID NO: 548 - protein, 18 aa, Artificial Sequence
  synthetic construct; peptide mimetic
DKWKAVYDKFAEAFREFF

SEQ ID NO: 549 - protein, 18 aa, Artificial Sequence
  synthetic construct; peptide mimetic
FFEKFAEAFKDYVAKWKD

SEQ ID NO: 550 - protein, 18 aa, Artificial Sequence
  synthetic construct; peptide mimetic
FFEKFAEAFKEYVAKWKE

SEQ ID NO: 551 - protein, 18 aa, Artificial Sequence
  synthetic construct; peptide mimetic
FFDKFADAFKDYVAKWKD

SEQ ID NO: 552 - protein, 18 aa, Artificial Sequence
  synthetic construct; peptide mimetic
FFERFAEAFKDYVAKWKD

SEQ ID NO: 553 - protein, 18 aa, Artificial Sequence
  synthetic construct; peptide mimetic
EFERFAEAFRDYVAKWKD

SEQ ID NO: 554 - protein, 18 aa, Artificial Sequence
  synthetic construct; peptide mimetic
FFEKFAEAFKDYVARWKD

SEQ ID NO: 555 - protein, 18 aa, Artificial Sequence
  synthetic construct; peptide mimetic
FFERFAEAFKDYVAKWRD

SEQ ID NO: 556 - protein, 18 aa, Artificial Sequence
  synthetic construct; peptide mimetic
FFDKFAEAFKDYVAKWKD

SEQ ID NO: 557 - protein, 18 aa, Artificial Sequence
  synthetic construct; peptide mimetic
FFEKFADAFKDYVAKWKD

SEQ ID NO: 558 - protein, 18 aa, Artificial Sequence
  synthetic construct; peptide mimetic
FFERFAEAFKEYVAKWKD

SEQ ID NO: 559 - protein, 18 aa, Artificial Sequence
  synthetic construct; peptide mimetic
FFERFAEAFKDYVAKWKE

SEQ ID NO: 560 - protein, 18 aa, Artificial Sequence
  synthetic construct; peptide mimetic
FFEKFKEFFKDYFAKFWD

SEQ ID NO: 561 - protein, 18 aa, Artificial Sequence
  synthetic construct; peptide mimetic
FFDKFKDFFKDYFAKFWD

SEQ ID NO: 562 - protein, 18 aa, Artificial Sequence
  synthetic construct; peptide mimetic
FFEKFKEFFKEYFAKFWE

SEQ ID NO: 563 - protein, 18 aa, Artificial Sequence
  synthetic construct; peptide mimetic
FFERFKEFFKDYFAKFWD

SEQ ID NO: 564 - protein, 18 aa, Artificial Sequence
  synthetic construct; peptide mimetic
FFEKFREFFKDYFAKFWD

SEQ ID NO: 565 - protein, 18 aa, Artificial Sequence
  synthetic construct; peptide mimetic
FFEKFKEFFRDYFAKFWD

SEQ ID NO: 566 - protein, 18 aa, Artificial Sequence
  synthetic construct; peptide mimetic
FFEKFKEFFKDYFARFWD

SEQ ID NO: 567 - protein, 18 aa, Artificial Sequence
  synthetic construct; peptide mimetic
FFDKFKEFFKDYFAKFWD

SEQ ID NO: 568 - protein, 18 aa, Artificial Sequence
  synthetic construct; peptide mimetic
FFEKFKDFFKDYFAKFWD

SEQ ID NO: 569 - protein, 18 aa, Artificial Sequence
  synthetic construct; peptide mimetic
FFEKFKEFFKEYFAKFWD

SEQ ID NO: 570 - protein, 18 aa, Artificial Sequence
  synthetic construct; peptide mimetic
FFEKFKEFFKDYFAKFWE

SEQ ID NO: 571 - protein, 18 aa, Artificial Sequence
  synthetic construct; epsilon-methylLys analog
  misc (4)..(4): Lys at position 4 is epsilon methylated
  misc (9)..(9): Lys at position 9 is epsilon methylated
  misc (13)..(13): Lys at position 13 is epsilon methylated
  misc (15)..(15): Lys at position 15 is epsilon methylated
DWFKAFYDKVAEKFKEAF

SEQ ID NO: 572 - protein, 18 aa, Artificial Sequence
  synthetic construct; epsilon-methylLys analog
  misc (4)..(4): Lys at position 4 is epsilon methylated
  misc (9)..(9): Lys at position 9 is epsilon methylated
  misc (13)..(13): Lys at position 13 is epsilon methylated
  misc (15)..(15): Lys at position 15 is epsilon methylated
DWFKAFYDKVAEKFKEAF

SEQ ID NO: 573 - protein, 18 aa, Artificial Sequence
  synthetic construct; epsilon-N-dimethylLys analog
  misc (4)..(4): Lys at position 4 is and epsilon-N-Dimethyl-Lys
  misc (9)..(9): Lys at position 9 is and epsilon-N-Dimethyl-Lys
  misc (13)..(13): Lys at position 9 is and epsilon-N-Dimethyl-Lys
  misc (15)..(15): Lys at position 9 is and epsilon-N-Dimethyl-Lys
DWFKAFYDKVAEKFKEAF

SEQ ID NO: 574 - protein, 18 aa, Artificial Sequence
  synthetic construct; epsilon-N-dimethylLys analog
  misc (4)..(4): Lys at position 4 is and epsilon-N-Dimethyl-Lys
  misc (9)..(9): Lys at position 9 is and epsilon-N-Dimethyl-Lys
  misc (13)..(13): Lys at position 13 is and epsilon-N-Dimethyl-Lys
  misc (15)..(15): Lys at position 15 is and epsilon-N-Dimethyl-Lys
DWFKAFYDKVAEKFKEAF

SEQ ID NO: 575 - protein, 18 aa, Artificial Sequence
  synthetic construct; epsilon-N-dimethylLys analog
  misc (4)..(4): Lys at position 4 is and epsilon-N-Dimethyl-Lys
  misc (9)..(9): Lys at position 9 is and epsilon-N-Dimethyl-Lys
DWFKAFYDKVAEKFKEAF

SEQ ID NO: 576 - protein, 18 aa, Artificial Sequence
  synthetic construct; epsilon-N-diethylLys analog
  misc (4)..(4): Lys at position 4 is and epsilon-N-Diethyl-Lys
  misc (9)..(9): Lys at position 9 is and epsilon-N-Diethyl-Lys
  misc (13)..(13): Lys at position 13 is and epsilon-N-Diethyl-Lys
  misc (15)..(15): Lys at position 15 is and epsilon-N-Diethyl-Lys
DWFKAFYDKVAEKFKEAF

SEQ ID NO: 577 - protein, 18 aa, Artificial Sequence
  synthetic construct; epsilon-N-diethylLys analog
  misc (4)..(4): Lys at position 4 is and epsilon-N-Diethyl-Lys
  misc (9)..(9): Lys at position 9 is and epsilon-N-Diethyl-Lys
  misc (13)..(13): Lys at position 13 is and epsilon-N-Diethyl-Lys
  misc (15)..(15): Lys at position 15 is and epsilon-N-Diethyl-Lys
DWFKAFYDKVAEKFKEAF

SEQ ID NO: 578 - protein, 18 aa, Artificial Sequence
  synthetic construct; epsilon-N-diethylLys analog
  misc (4)..(4): Lys at position 4 is and epsilon-N-Diethyl-Lys
  misc (9)..(9): Lys at position 9 is and epsilon-N-Diethyl-Lys
  misc (13)..(13): Lys at position 13 is and epsilon-N-Diethyl-Lys
  misc (13)..(13): Lys at position 15 is and epsilon-N-Diethyl-Lys
DWFKAFYDKVAEKFKEAF

SEQ ID NO: 579 - protein, 18 aa, Artificial Sequence
  synthetic construct; epsilon-N-monomethylLys analog
  misc (4)..(4): Lys at position 4 is and epsilon-N-monomethyl-Lys
  misc (9)..(9): Lys at position 9 is and epsilon-N-monomiethyl-Lys
  misc (13)..(13): Lys at position 13 is and epsilon-N-monomethyl-Lys
  misc (15)..(15): Lys at position 15 is and epsilon-N-monomethyl-Lys
DWFKAFYDKVAEKFKEAF

SEQ ID NO: 580 - protein, 18 aa, Artificial Sequence
  synthetic construct; epsilon-N-monomethylLys analog
  misc (4)..(4): Lys at position 4 is and epsilon-N-monomethyl-Lys
  misc (9)..(9): Lys at position 9 is and epsilon-N-monomethyl-Lys
  misc (13)..(13): Lys at position 13 is and epsilon-N-monomethyl-Lys
  misc (15)..(15): Lys at position 15 is and epsilon-N-monomethyl-Lys
DWFKAFYDKVAEKFKEAF

SEQ ID NO: 581 - protein, 18 aa, Artificial Sequence
  synthetic construct; epsilon-N-monomethylLys analog
  misc (4)..(4): Lys at position 4 is and epsilon-N-monomethyl-Lys
  misc (9)..(9): Lys at position 9 is and epsilon-N-monomethyl-Lys
  misc (13)..(13): Lys at position 13 is and epsilon-N-monomethyl-Lys
  misc (15)..(15): Lys at position 15 is and epsilon-N-monomethyl-Lys
DWFKAFYDKVAEKFKEAF

SEQ ID NO: 582 - protein, 18 aa, Artificial Sequence
  synthetic construct; epsilon-N-ethylLys analog
  misc (4)..(4): Lys at position 4 is and epsilon-N-ethyl-Lys
  misc (9)..(9): Lys at position 9 is and epsilon-N-ethyl-Lys
  misc (13)..(13): Lys at position 13 is and epsilon-N-ethyl-Lys
  misc (15)..(15): Lys at position 15 is and epsilon-N-ethyl-Lys
DWFKAFYDKVAEKFKEAF

SEQ ID NO: 583 - protein, 18 aa, Artificial Sequence
  synthetic construct; epsilon-N-ethylLys analog
  misc (4)..(4): Lys at position 4 is and epsilon-N-ethyl-Lys
  misc (9)..(9): Lys at position 9 is and epsilon-N-ethyl-Lys
  misc (13)..(13): Lys at position 13 is and epsilon-N-ethyl-Lys
  misc (15)..(15): Lys at position 15 is and epsilon-N-ethyl-Lys
DWFKAFYDKVAEKFKEAF

SEQ ID NO: 584 - protein, 18 aa, Artificial Sequence
  synthetic construct; epsilon-N-ethylLys analog
  misc (4)..(4): Lys at position 4 is and epsilon-N-ethyl-Lys
  misc (9)..(9): Lys at position 9 is and epsilon-N-ethyl-Lys
  misc (13)..(13): Lys at position 13 is and epsilon-N-ethyl-Lys
  misc (15)..(15): Lys at position 15 is and epsilon-N-ethyl-Lys
DWFKAFYDKVAEKFKEAF

SEQ ID NO: 585 - protein, 18 aa, Artificial Sequence
  synthetic construct; homoLys analog
  misc (4)..(4): Lys at position 4 is a homoLys
  misc (9)..(9): Lys at position 9 is a homoLys
  misc (13)..(13): Lys at position 13 is a homoLys
  misc (15)..(15): Lys at position 15 is a homoLys
DWFKAFYDKVAEKFKEAF

SEQ ID NO: 586 - protein, 18 aa, Artificial Sequence
  synthetic construct; homoLys analog
  misc (4)..(4): Lys at position 4 is homoLys
  misc (9)..(9): Lys at position 9 is homoLys
  misc (13)..(13): Lys at position 13 is homoLys
  misc (15)..(15): Lys at position 15 is homoLys
DWFKAFYDKVAEKFKEAF

SEQ ID NO: 587 - protein, 18 aa, Artificial Sequence
  synthetic construct; homoLys analog
  misc (4)..(4): Lys at position 4 is homoLys
  misc (9)..(9): Lys at position 9 is homoLys
  misc (13)..(13): Lys at position 13 is homoLys
  misc (15)..(15): Lys at position 13 is homoLys
DWFKAFYDKVAEKFKEAF

SEQ ID NO: 588 - protein, 18 aa, Artificial Sequence
  synthetic construct; homoLys analog
  misc (4)..(4): Lys at position 4 is homoLys
  misc (9)..(9): Lys at position 9 is homoLys
  misc (13)..(13): Lys at position 13 is homoLys
  misc (15)..(15): Lys at position 15 is homoLys
DWFKAFYDKVAEKFKEAF

SEQ ID NO: 589 - protein, 18 aa, Artificial Sequence
  synthetic construct; homoLys analog
  misc (4)..(4): Lys at position 4 is homoLys
  misc (9)..(9): Lys at position 9 is homoLys
  misc (13)..(13): Lys at position 13 is homoLys
  misc (15)..(15): Lys at position 15 is homoLys
DWFKAFYDKVAEKFKEAF

SEQ ID NO: 590 - protein, 18 aa, Artificial Sequence
  synthetic construct; homoLys analog
  misc (4)..(4): Lys at position 4 is homoLys
  misc (9)..(9): Lys at position 9 is homoLys
  misc (13)..(13): Lys at position 13 is homoLys
  misc (15)..(15): Lys at position 15 is homoLys
DWFKAFYDKVAEKFKEAF

SEQ ID NO: 591 - protein, 18 aa, Artificial Sequence
  synthetic construct; homoLys analog
  misc (4)..(4): Lys at position 4 is homoLys
  misc (9)..(9): Lys at position 9 is homoLys
  misc (13)..(13): Lys at position 13 is homoLys
  misc (15)..(15): Lys at position 15 is homoLys
DWFKAFYDKVAEKFKEAF

SEQ ID NO: 592 - protein, 18 aa, Artificial Sequence
  synthetic construct; homoLys analog
  misc (4)..(4): Lys at position 4 is homoLys
  misc (9)..(9): Lys at position 9 is homoLys
  misc (13)..(13): Lys at position 13 is homoLys
  misc (15)..(15): Lys at position 15 is homoLys
DWFKAFYDKVAEKFKEAF

SEQ ID NO: 593 - protein, 18 aa, Artificial Sequence
  synthetic construct; homoLys analog
  misc (4)..(4): Lys at position 4 is homoLys
  misc (9)..(9): Lys at position 9 is homoLys
  misc (13)..(13): Lys at position 13 is homoLys
  misc (15)..(15): Lys at position 15 is homoLys
DWFKAFYDKVAEKFKEAF

SEQ ID NO: 594 - protein, 18 aa, Artificial Sequence
  synthetic construct; homoLys analog
  misc (4)..(4): Lys at position 4 is homoLys
  misc (9)..(9): Lys at position 9 is homoLys
  misc (13)..(13): Lys at position 13 is homoLys
  misc (15)..(15): Lys at position 15 is homoLys
DWFKAFYDKVAEKFKEAF

SEQ ID NO: 595 - protein, 18 aa, Artificial Sequence
  synthetic construct; homoLys analog
  misc (4)..(4): Lys at position 4 is homoLys
  misc (9)..(9): Lys at position 9 is homoLys
  misc (13)..(13): Lys at position 13 is homoLys
  misc (15)..(15): Lys at position 15 is homoLys
DWFKAFYDKVAEKFKEAF

SEQ ID NO: 596 - protein, 18 aa, Artificial Sequence
  synthetic construct; ornithine analogs
  misc (4)..(4): Xaa at position 4 is a delta-N-dimethyl-ornithine
  misc (9)..(9): Xaa at position 9 is a delta-N-dimethyl-ornithine
  misc (13)..(13): Xaa at position 13 is a delta-N-dimethyl-ornithine
  misc (15)..(15): Xaa at position 15 is a delta-N-dimethyl-ornithine
DWFXAFYDXVAEXFXEAF

SEQ ID NO: 597 - protein, 18 aa, Artificial Sequence
  synthetic construct; ornithine analogs
  misc (4)..(4): Xaa at position 4 is a delta-N-dimethyl-ornithine
  misc (9)..(9): Xaa at position 9 is a delta-N-dimethyl-ornithine
  misc (13)..(13): Xaa at position 13 is a delta-N-dimethyl-ornithine
  misc (15)..(15): Xaa at position 15 is a delta-N-dimethyl-ornithine
DWFXAFYDXVAEXFXEAF

SEQ ID NO: 598 - protein, 18 aa, Artificial Sequence
  synthetic construct; ornithine analogs
  misc (4)..(4): Xaa at position 4 is a delta-N-dimethyl-ornithine
  misc (9)..(9): Xaa at position 9 is a delta-N-dimethyl-ornithine
  misc (13)..(13): Xaa at position 13 is a delta-N-dimethyl-ornithine
  misc (15)..(15): Xaa at position 15 is a delta-N-dimethyl-ornithine
DWFXAFYDXVAEXFXEAF

SEQ ID NO: 599 - protein, 18 aa, Artificial Sequence
  synthetic construct; ornithine analogs
  misc (4)..(4): Xaa at position 4 is a delta-N-dimethyl-ornithine
  misc (9)..(9): Xaa at position 9 is a delta-N-dimethyl-ornithine
  misc (13)..(13): Xaa at position 13 is a delta-N-dimethyl-ornithine
  misc (15)..(15): Xaa at position 15 is a delta-N-dimethyl-ornithine
DWFXAFYDXVAEXFXEAF

SEQ ID NO: 600 - protein, 18 aa, Artificial Sequence
  synthetic construct; ornithine analogs
  misc (4)..(4): Xaa at position 4 is a delta-N-diethyl-ornithine
  misc (9)..(9): Xaa at position 9 is a delta-N-diethyl-ornithine
  misc (13)..(13): Xaa at position 13 is a delta-N-diethyl-ornithine
  misc (15)..(15): Xaa at position 15 is a delta-N-diethyl-ornithine
DWFXAFYDXVAEXFXEAF

SEQ ID NO: 601 - protein, 18 aa, Artificial Sequence
  synthetic construct; ornithine analogs
  misc (4)..(4): Xaa at position 4 is a delta-N-methyl-ornithine
  misc (9)..(9): Xaa at position 9 is a delta-N-methyl-ornithine
  misc (13)..(13): Xaa at position 13 is a delta-N-methyl-ornithine
  misc (15)..(15): Xaa at position 15 is a delta-N-methyl-ornithine
DWFXAFYDXVAEXFXEAF

SEQ ID NO: 602 - protein, 18 aa, Artificial Sequence
  synthetic construct; ornithine analogs
  misc (4)..(4): Xaa at position 4 is a delta-N-methyl-ornithine
  misc (9)..(9): Xaa at position 9 is a delta-N-methyl-ornithine
  misc (13)..(13): Xaa at position 13 is a delta-N-methyl-ornithine
  misc (15)..(15): Xaa at position 15 is a delta-N-methyl-ornithine
DWFXAFYDXVAEXFXEAF

SEQ ID NO: 603 - protein, 18 aa, Artificial Sequence
  synthetic construct; ornithine analogs
  misc (4)..(4): Xaa at position 4 is a delta-N-methyl-ornithine
  misc (9)..(9): Xaa at position 9 is a delta-N-methyl-ornithine
  misc (13)..(13): Xaa at position 13 is a delta-N-methyl-ornithine
  misc (15)..(15): Xaa at position 15 is a delta-N-methyl-ornithine
DWFXAFYDXVAEXFXEAF

SEQ ID NO: 604 - protein, 18 aa, Artificial Sequence
  synthetic construct; ornithine analogs
  misc (4)..(4): Xaa at position 4 is a delta-N-ethyl-ornithine
  misc (9)..(9): Xaa at position 9 is a delta-N-ethyl-ornithine
  misc (13)..(13): Xaa at position 13 is a delta-N-ethyl-ornithine
  misc (15)..(15): Xaa at position 15 is a delta-N-ethyl-ornithine
DWFXAFYDXVAEXFXEAF

SEQ ID NO: 605 - protein, 18 aa, Artificial Sequence
  synthetic construct; ornithine analogs
  misc (4)..(4): Xaa at position 4 is a delta-N-ethyl-ornithine
  misc (9)..(9): Xaa at position 9 is a delta-N-ethyl-ornithine
  misc (13)..(13): Xaa at position 13 is a delta-N-ethyl-ornithine
  misc (15)..(15): Xaa at position 15 is a delta-N-ethyl-ornithine
DWFXAFYDXVAEXFXEAF

SEQ ID NO: 606 - protein, 18 aa, Artificial Sequence
  synthetic construct; ornithine analogs
  misc (4)..(4): Xaa at position 4 is a delta-N-ethyl-ornithine
  misc (9)..(9): Xaa at position 9 is a delta-N-ethyl-ornithine
  misc (13)..(13): Xaa at position 13 is a delta-N-ethyl-ornithine
  misc (15)..(15): Xaa at position 15 is a delta-N-ethyl-ornithine
DWFXAFYDXVAEXFXEAF

SEQ ID NO: 607 - protein, 10 aa, Artificial Sequence
  synthetic construct; receptor binding domains of ApoE
RLLRKRLKRL

SEQ ID NO: 608 - protein, 10 aa, Artificial Sequence
  synthetic construct; receptor binding domain of ApoE
RMLRKRMKRL

SEQ ID NO: 609 - protein, 10 aa, Artificial Sequence
  synthetic construct; receptor binding domain of ApoE
RLLRKPLKRL

SEQ ID NO: 610 - protein, 10 aa, Artificial Sequence
  synthetic construct; receptor binding domain of ApoE
RVLRKRVNRL

SEQ ID NO: 611 - protein, 10 aa, Artificial Sequence
  synthetic construct; receptor binding domain of ApoE
RLVRKRLKRM

SEQ ID NO: 612 - protein, 10 aa, Artificial Sequence
  synthetic construct; receptor binding domain of ApoE
RLLRRRLRRL

SEQ ID NO: 613 - protein, 10 aa, Artificial Sequence
  synthetic construct; receptor binding domain of ApoE
RFFRKRLKRL

SEQ ID NO: 614 - protein, 18 aa, Artificial Sequence
  synthetic construct; Lipid-Associating Peptide
FAEKLKEAVKDYFAKLWD

SEQ ID NO: 615 - protein, 18 aa, Artificial Sequence
  synthetic construct; Lipid-Associating Peptide
FAEKFKEAVKDYFAKFWD

SEQ ID NO: 616 - protein, 18 aa, Artificial Sequence
  synthetic construct; peptide mimetic
DWLKAFYDKVFEKFKEAF

SEQ ID NO: 617 - protein, 18 aa, Artificial Sequence
  synthetic construct; peptide mimetic
DWLKAFYDKVAEKFKEFF

SEQ ID NO: 618 - protein, 18 aa, Artificial Sequence
  synthetic construct; lipid-associating peptide
DWLRAFYDKVAEKLREAF

SEQ ID NO: 619 - protein, 18 aa, Artificial Sequence
  synthetic construct; lipid associating peptide
DWLRALYDKVAEKLREAL

SEQ ID NO: 620 - protein, 18 aa, Artificial Sequence
  synthetic construct; lipid associating peptide
DLLRALYDKVAEKLREAW

SEQ ID NO: 621 - protein, 10 aa, Artificial Sequence
  synthetic construct; Rat ApoE mimetic
LRRMRRRLMR

SEQ ID NO: 622 - protein, 8 aa, Artificial Sequence
  synthetic construct; Rat ApoE mimetic
RLTRRRGK

SEQ ID NO: 623 - protein, 28 aa, Artificial Sequence
  synthetic construct; ApoE-mimicking peptide
  MISC_FEATURE (1)..(1): N-terminal butanoyl
LRRLRRRLLRDWLKAFYDKVAEKLKEAF

SEQ ID NO: 624 - protein, 28 aa, Artificial Sequence
  synthetic construct; ApoE mimicking peptide
  MISC_FEATURE (1)..(1): N-terminal hexanoyl
LRRLRRRLLRDWLKAFYDKVAEKLKEAF

SEQ ID NO: 625 - protein, 28 aa, Artificial Sequence
  synthetic construct; ApoE mimicking peptide
  MISC_FEATURE (1)..(1): N-terminal octanoyl
LRRLRRRLLRDWLKAFYDKVAEKLKEAF

SEQ ID NO: 626 - protein, 28 aa, Artificial Sequence
  synthetic construct; ApoE mimicking peptide
  MISC_FEATURE (1)..(1): N-terminal decanoyl
LRRLRRRLLRDWLKAFYDKVAEKLKEAF

SEQ ID NO: 627 - protein, 28 aa, Artificial Sequence
  synthetic construct; ApoE mimicking peptide
  MISC_FEATURE (1)..(1): N-terminal lauroyl
LRRLRRRLLRDWLKAFYDKVAEKLKEAF

SEQ ID NO: 628 - protein, 28 aa, Artificial Sequence
  synthetic construct; ApoE mimicking peptide
  MISC_FEATURE (1)..(1): N-terminal myristoyl
LRRLRRRLLRDWLKAFYDKVAEKLKEAF

SEQ ID NO: 629 - protein, 28 aa, Artificial Sequence
  synthetic construct; ApoE mimicking peptide
  MISC_FEATURE (1)..(1): N-terminal palmitoyl
LRRLRRRLLRDWLKAFYDKVAEKLKEAF

SEQ ID NO: 630 - protein, 28 aa, Artificial Sequence
  synthetic construct; ApoE mimicking peptide
  MISC_FEATURE (1)..(1): N-terminal stearoyl
LRRLRRRLLRDWLKAFYDKVAEKLKEAF

SEQ ID NO: 631 - protein, 28 aa, Artificial Sequence
  synthetic construct; ApoE mimicking peptide
  MISC_FEATURE (1)..(1): N-terminal palmitoleoyl
LRRLRRRLLRDWLKAFYDKVAEKLKEAF

SEQ ID NO: 632 - protein, 28 aa, Artificial Sequence
  synthetic construct; ApoE mimicking peptide
  MISC_FEATURE (1)..(1): N-terminal arachidoyl
LRRLRRRLLRDWLKAFYDKVAEKLKEAF

SEQ ID NO: 633 - protein, 28 aa, Artificial Sequence
  synthetic construct; ApoE mimicking peptide
  MISC_FEATURE (1)..(1): N-terminal behenoyl
LRRLRRRLLRDWLKAFYDKVAEKLKEAF

SEQ ID NO: 634 - protein, 28 aa, Artificial Sequence
  synthetic construct; ApoE mimicking peptide
  MISC_FEATURE (1)..(1): N-terminal oleoyl
LRRLRRRLLRDWLKAFYDKVAEKLKEAF

SEQ ID NO: 635 - protein, 28 aa, Artificial Sequence
  synthetic construct; ApoE mimicking peptide
  MISC_FEATURE (1)..(1): N-terminal ricinoleoyl
LRRLRRRLLRDWLKAFYDKVAEKLKEAF

SEQ ID NO: 636 - protein, 28 aa, Artificial Sequence
  synthetic construct; ApoE mimicking peptide
  MISC_FEATURE (1)..(1): N-terminal linolenoyl
LRRLRRRLLRDWLKAFYDKVAEKLKEAF

SEQ ID NO: 637 - protein, 28 aa, Artificial Sequence
  synthetic construct; ApoE mimicking peptide
  MISC_FEATURE (1)..(1): N-terminal vacceoyl
LRRLRRRLLRDWLKAFYDKVAEKLKEAF

SEQ ID NO: 638 - protein, 28 aa, Artificial Sequence
  synthetic construct; ApoE mimicking peptide
  MISC_FEATURE (1)..(1): N-terminal gadoleoyl
LRRLRRRLLRDWLKAFYDKVAEKLKEAF

SEQ ID NO: 639 - protein, 28 aa, Artificial Sequence
  synthetic construct; ApoE mimicking peptide
  MISC_FEATURE (1)..(1): N-terminal erucoyl
LRRLRRRLLRDWLKAFYDKVAEKLKEAF

SEQ ID NO: 640 - protein, 28 aa, Artificial Sequence
  synthetic construct; ApoE mimicking peptide
  MISC_FEATURE (1)..(1): N-terminal cetoleoyl
LRRLRRRLLRDWLKAFYDKVAEKLKEAF

SEQ ID NO: 641 - protein, 28 aa, Artificial Sequence
  synthetic construct; ApoE mimicking peptide
  MISC_FEATURE (1)..(1): N-terminal nervonoyl
LRRLRRRLLRDWLKAFYDKVAEKLKEAF

SEQ ID NO: 642 - protein, 28 aa, Artificial Sequence
  synthetic construct; ApoE mimicking peptide
  MISC_FEATURE (1)..(1): N-terminal adrenoyl
LRRLRRRLLRDWLKAFYDKVAEKLKEAF

SEQ ID NO: 643 - protein, 28 aa, Artificial Sequence
  synthetic construct; ApoE mimicking peptide
  MISC_FEATURE (1)..(1): N-terminal alpha-linolenoyl
LRRLRRRLLRDWLKAFYDKVAEKLKEAF

SEQ ID NO: 644 - protein, 28 aa, Artificial Sequence
  synthetic construct; ApoE mimicking peptide
  MISC_FEATURE (1)..(1): N-terminal gamma-linolenoyl
LRRLRRRLLRDWLKAFYDKVAEKLKEAF

SEQ ID NO: 645 - protein, 28 aa, Artificial Sequence
  synthetic construct; ApoE mimicking peptide
  MISC_FEATURE (1)..(1): N-terminal EPA
LRRLRRRLLRDWLKAFYDKVAEKLKEAF

SEQ ID NO: 646 - protein, 28 aa, Artificial Sequence
  synthetic construct; ApoE mimicking peptide
  MISC_FEATURE (1)..(1): N-terminal DHA
LRRLRRRLLRDWLKAFYDKVAEKLKEAF

SEQ ID NO: 647 - protein, 28 aa, Artificial Sequence
  synthetic construct; ApoE mimicking peptide
  MISC_FEATURE (1)..(1): N-terminal fish oil
LRRLRRRLLRDWLKAFYDKVAEKLKEAF

SEQ ID NO: 648 - protein, 28 aa, Artificial Sequence
  synthetic construct; ApoE mimicking peptide
  MISC_FEATURE (1)..(1): N-terminal 4-amino-butanoyl
LRRLRRRLLRDWLKAFYDKVAEKLKEAF

SEQ ID NO: 649 - protein, 28 aa, Artificial Sequence
  synthetic construct; ApoE mimicking peptide
  MISC_FEATURE (1)..(1): N-terminal 6-amino-hexanoyl
LRRLRRRLLRDWLKAFYDKVAEKLKEAF

SEQ ID NO: 650 - protein, 28 aa, Artificial Sequence
  synthetic construct; ApoE mimicking peptide
  MISC_FEATURE (1)..(1): N-terminal 8-amino-octanoyl
LRRLRRRLLRDWLKAFYDKVAEKLKEAF

SEQ ID NO: 651 - protein, 28 aa, Artificial Sequence
  synthetic construct; ApoE mimicking peptide
  MISC_FEATURE (1)..(1): N-terminal 10-amino-decanoyl
LRRLRRRLLRDWLKAFYDKVAEKLKEAF

SEQ ID NO: 652 - protein, 28 aa, Artificial Sequence
  synthetic construct; ApoE mimicking peptide
  MISC_FEATURE (1)..(1): N-terminal 12-amino-lauroyl
LRRLRRRLLRDWLKAFYDKVAEKLKEAF

SEQ ID NO: 653 - protein, 28 aa, Artificial Sequence
  synthetic construct; ApoE mimicking peptide
  MISC_FEATURE (1)..(1): N-terminal 14-amino-myristoyl
LRRLRRRLLRDWLKAFYDKVAEKLKEAF

SEQ ID NO: 654 - protein, 28 aa, Artificial Sequence
  synthetic construct; ApoE mimicking peptide
  MISC_FEATURE (1)..(1): N-terminal 16-amino-palmitoyl
LRRLRRRLLRDWLKAFYDKVAEKLKEAF

SEQ ID NO: 655 - protein, 28 aa, Artificial Sequence
  synthetic construct; ApoE mimicking peptide
  MISC_FEATURE (1)..(1): N-terminal 16-amino-palmitoleoyl
LRRLRRRLLRDWLKAFYDKVAEKLKEAF

SEQ ID NO: 656 - protein, 28 aa, Artificial Sequence
  synthetic construct; ApoE mimicking peptide
  MISC_FEATURE (1)..(1): N-terminal 18-amino-stearoyl
LRRLRRRLLRDWLKAFYDKVAEKLKEAF

SEQ ID NO: 657 - protein, 28 aa, Artificial Sequence
  synthetic construct; ApoE mimicking peptide
  MISC_FEATURE (1)..(1): N-terminal 18-amino-oleoyl
LRRLRRRLLRDWLKAFYDKVAEKLKEAF

SEQ ID NO: 658 - protein, 28 aa, Artificial Sequence
  synthetic construct; ApoE mimicking peptide
  MISC_FEATURE (1)..(1): N-terminal 18-amino-linolenoyl
LRRLRRRLLRDWLKAFYDKVAEKLKEAF

SEQ ID NO: 659 - protein, 28 aa, Artificial Sequence
  synthetic construct; ApoE mimicking peptide
  MISC_FEATURE (1)..(1): N-terminal 20-amino-arachidoyl
LRRLRRRLLRDWLKAFYDKVAEKLKEAF

SEQ ID NO: 660 - protein, 18 aa, Artificial Sequence
  synthetic construct; lipid associating peptide
KAFEEVLAKKFYDKALWD

SEQ ID NO: 661 - protein, 10 aa, Artificial Sequence
  synthetic construct; receptor binding domain of Apo E
LRLLRKLKRR